European Patent Specification EP 3 981 792 B1, published August 21, 2024. Title: PD-1-Binding Molecules and Methods of Use Thereof. Applicant: MacroGenic, Inc. Shah, Kalpana Smith, Douglas La Motte-Mohs, Ross Johnson, Leslie Moore, Paul Bonvini, Ezio Koenig, Scott. The sequence listing filed with the application follows.

SEQUENCE LISTING (298 sequences)

SEQ ID NO: 1 - protein, 217 aa, Homo sapiens
  MISC_FEATURE (1)..(217): Human IgG1 CH2-CH3 Domain
  MISC_FEATURE (217)..(217): Xaa is a lysine (K) or is absent
APELLGGPSVFLFPPKPKDTLMISRTPEVTCVVVDVSHEDPEVKFNWYVDGVEVHNAKTKPREEQYNSTYRVVSVLTVLHQDWLNGKEYKCKVSNKALPAPIEKTISKAKGQPREPQVYTLPPSREEMTKNQVSLTCLVKGFYPSDIAVEWESNGQPENNYKTTPPVLDSDGSFFLYSKLTVDKSRWQQGNVFSCSVMHEALHNHYTQKSLSLSPGX

SEQ ID NO: 2 - protein, 216 aa, Homo sapiens
  MISC_FEATURE (1)..(216): Human IgG2 CH2-CH3 Domain
  MISC_FEATURE (216)..(216): Xaa is a lysine (K) or is absent
APPVAGPSVFLFPPKPKDTLMISRTPEVTCVVVDVSHEDPEVQFNWYVDGVEVHNAKTKPREEQFNSTFRVVSVLTVVHQDWLNGKEYKCKVSNKGLPAPIEKTISKTKGQPREPQVYTLPPSREEMTKNQVSLTCLVKGFYPSDISVEWESNGQPENNYKTTPPMLDSDGSFFLYSKLTVDKSRWQQGNVFSCSVMHEALHNHYTQKSLSLSPGX

SEQ ID NO: 3 - protein, 217 aa, Homo sapiens
  MISC_FEATURE (1)..(217): Human IgG3 CH2-CH3 Domain
  MISC_FEATURE (217)..(217): Xaa is a lysine (K) or is absent
APELLGGPSVFLFPPKPKDTLMISRTPEVTCVVVDVSHEDPEVQFKWYVDGVEVHNAKTKPREEQYNSTFRVVSVLTVLHQDWLNGKEYKCKVSNKALPAPIEKTISKTKGQPREPQVYTLPPSREEMTKNQVSLTCLVKGFYPSDIAVEWESSGQPENNYNTTPPMLDSDGSFFLYSKLTVDKSRWQQGNIFSCSVMHEALHNRFTQKSLSLSPGX

SEQ ID NO: 4 - protein, 217 aa, Homo sapiens
  MISC_FEATURE (1)..(217): Human IgG4 CH2-CH3 Domain
  MISC_FEATURE (217)..(217): Xaa is a lysine (K) or is absent
APEFLGGPSVFLFPPKPKDTLMISRTPEVTCVVVDVSQEDPEVQFNWYVDGVEVHNAKTKPREEQFNSTYRVVSVLTVLHQDWLNGKEYKCKVSNKGLPSSIEKTISKAKGQPREPQVYTLPPSQEEMTKNQVSLTCLVKGFYPSDIAVEWESNGQPENNYKTTPPVLDSDGSFFLYSRLTVDKSRWQEGNVFSCSVMHEALHNHYTQKSLSLSLGX

SEQ ID NO: 5 - protein, 217 aa, Artificial Sequence
  Human IgG1 CH2-CH3 Domain Having L234A/L235A Substitutions
  MISC_FEATURE (217)..(217): Xaa is a lysine (K) or is absent
APEAAGGPSVFLFPPKPKDTLMISRTPEVTCVVVDVSHEDPEVKFNWYVDGVEVHNAKTKPREEQYNSTYRVVSVLTVLHQDWLNGKEYKCKVSNKALPAPIEKTISKAKGQPREPQVYTLPPSREEMTKNQVSLTCLVKGFYPSDIAVEWESNGQPENNYKTTPPVLDSDGSFFLYSKLTVDKSRWQQGNVFSCSVMHEALHNHYTQKSLSLSPGX

SEQ ID NO: 6 - protein, 217 aa, Artificial Sequence
  "Knob-Bearing" Human IgG1 CH2-CH3 Domain
  MISC_FEATURE (217)..(217): Xaa is a lysine (K) or is absent
APEAAGGPSVFLFPPKPKDTLMISRTPEVTCVVVDVSHEDPEVKFNWYVDGVEVHNAKTKPREEQYNSTYRVVSVLTVLHQDWLNGKEYKCKVSNKALPAPIEKTISKAKGQPREPQVYTLPPSREEMTKNQVSLWCLVKGFYPSDIAVEWESNGQPENNYKTTPPVLDSDGSFFLYSKLTVDKSRWQQGNVFSCSVMHEALHNHYTQKSLSLSPGX

SEQ ID NO: 7 - protein, 217 aa, Artificial Sequence
  "Hole-Bearing" Human IgG1 CH2-CH3 Domain
  MISC_FEATURE (217)..(217): Xaa is a lysine (K) or is absent
APEAAGGPSVFLFPPKPKDTLMISRTPEVTCVVVDVSHEDPEVKFNWYVDGVEVHNAKTKPREEQYNSTYRVVSVLTVLHQDWLNGKEYKCKVSNKALPAPIEKTISKAKGQPREPQVYTLPPSREEMTKNQVSLSCAVKGFYPSDIAVEWESNGQPENNYKTTPPVLDSDGSFFLVSKLTVDKSRWQQGNVFSCSVMHEALHNRYTQKSLSLSPGX

SEQ ID NO: 8 - protein, 107 aa, Homo sapiens [sequence omitted]

SEQ ID NO: 9 - protein, 104 aa, Homo sapiens
  MISC_FEATURE (1)..(104): Human IgG CL Lambda Domain
QPKAAPSVTLFPPSSEELQANKATLVCLISDFYPGAVTVAWKADSSPVKAGVETTPSKQSNNKYAASSYLSLTPEQWKSHRSYSCQVTHEGSTVEKTVAPTECS

SEQ ID NO: 10 - protein, 98 aa, Homo sapiens
  MISC_FEATURE (1)..(98): Human IgG1 CH1 Domain
ASTKGPSVFPLAPSSKSTSGGTAALGCLVKDYFPEPVTVSWNSGALTSGVHTFPAVLQSSGLYSLSSVVTVPSSSLGTQTYICNVNHKPSNTKVDKRV

SEQ ID NO: 11 - protein, 12 aa, Homo sapiens
  MISC_FEATURE (1)..(12): Human IgG2 Hinge Region
ERKCCVECPPCP

SEQ ID NO: 12 - protein, 12 aa, Homo sapiens
  MISC_FEATURE (1)..(12): Human IgG4 Hinge Region
ESKYGPPCPSCP

SEQ ID NO: 13 - protein, 12 aa, Artificial Sequence
  Stabilized IgG4 Hinge Region
ESKYGPPCPPCP

SEQ ID NO: 14 - protein, 8 aa, Artificial Sequence
  Linker 1
GGGSGGGG

SEQ ID NO: 15 - protein, 6 aa, Artificial Sequence
  Cysteine-containing Linker 2
GGCGGG

SEQ ID NO: 16 - protein, 7 aa, Artificial Sequence
  Heterodimer-Promoting Domain
GVEPKSC

SEQ ID NO: 17 - protein, 6 aa, Artificial Sequence
  Heterodimer-Promoting Domain
VEPKSC

SEQ ID NO: 18 - protein, 6 aa, Artificial Sequence
  Heterodimer-Promoting Domain
AEPKSC

SEQ ID NO: 19 - protein, 7 aa, Artificial Sequence
  Heterodimer-Promoting Domain
GFNRGEC

SEQ ID NO: 20 - protein, 6 aa, Artificial Sequence
  Heterodimer-Promoting Domain
FNRGEC

SEQ ID NO: 21 - protein, 28 aa, Artificial Sequence
  Heterodimer-Promoting (E-coil) Domain
EVAALEKEVAALEKEVAALEKEVAALEK

SEQ ID NO: 22 - protein, 28 aa, Artificial Sequence
  Heterodimer-Promoting "K-coil" Domain
KVAALKEKVAALKEKVAALKEKVAALKE

SEQ ID NO: 23 - protein, 28 aa, Artificial Sequence
  Cysteine-Containing Heterodimer-Promoting "E-coil" Domain
EVAACEKEVAALEKEVAALEKEVAALEK

SEQ ID NO: 24 - protein, 28 aa, Artificial Sequence
  Cysteine-Containing Heterodimer-Promoting "K-coil" Domain
KVAACKEKVAALKEKVAALKEKVAALKE

SEQ ID NO: 25 - protein, 46 aa, Streptococcus dysgalactiae
  MISC_FEATURE (1)..(46): Albumin-Binding Domain 3 of Protein G of Streptococcus Strain G148
LAEAKVLANRELDKYGVSDYYKNLIDNAKSAEGVKALIDEILAALP

SEQ ID NO: 26 - protein, 46 aa, Artificial Sequence; identical to SEQ ID NO: 25
  Variant deimmunized Albumin Binding Domain

SEQ ID NO: 27 - protein, 46 aa, Artificial Sequence
  Variant Deimmunized Albumin Binding Domain
LAEAKVLANRELDKYGVSDYYKNAANNAKTVEGVKALIAEILAALP

SEQ ID NO: 28 - protein, 46 aa, Artificial Sequence
  Variant deimmunized Albumin Binding Domain
LAEAKVLANRELDKYGVSDYYKNLISNAKSVEGVKALIAEILAALP

SEQ ID NO: 29 - protein, 4 aa, Artificial Sequence
  Alternative Linker 2
GGGS

SEQ ID NO: 30 - protein, 5 aa, Artificial Sequence
  Alternative Linker 2
ASTKG

SEQ ID NO: 31 - protein, 10 aa, Artificial Sequence
  Linker
DKTHTCPPCP

SEQ ID NO: 32 - protein, 15 aa, Artificial Sequence
  Linker
EPKSCDKTHTCPPCP

SEQ ID NO: 33 - protein, 6 aa, Artificial Sequence
  Alternative Linker 2
LEPKSS

SEQ ID NO: 34 - protein, 5 aa, Artificial Sequence
  Alternative Linker 2
APSSS

SEQ ID NO: 35 - protein, 8 aa, Artificial Sequence
  Linker
APSSSPME

SEQ ID NO: 36 - protein, 15 aa, Artificial Sequence
  Linker
LEPKSADKTHTCPPC

SEQ ID NO: 37 - protein, 16 aa, Artificial Sequence
  Linker
LEPKSSDKTHTCPPCP

SEQ ID NO: 38 - protein, 525 aa, Homo sapiens
  MISC_FEATURE (1)..(525): Human LAG-3 (Signaling Sequence and Mature Protein)
  MISC_FEATURE (1)..(28): Signaling Sequence
  MISC_FEATURE (29)..(525): Mature Protein
MWEAQFLGLLFLQPLWVAPVKPLQPGAEVPVVWAQEGAPAQLPCSPTIPLQDLSLLRRAGVTWQHQPDSGPPAAAPGHPLAPGPHPAAPSSWGPRPRRYTVLSVGPGGLRSGRLPLQPRVQLDERGRQRGDFSLWLRPARRADAGEYRAAVHLRDRALSCRLRLRLGQASMTASPPGSLRASDWVILNCSFSRPDRPASVHWFRNRGQGRVPVRESPHHHLAESFLFLPQVSPMDSGPWGCILTYRDGFNVSIMYNLTVLGLEPPTPLTVYAGAGSRVGLPCRLPAGVGTRSFLTAKWTPPGGGPDLLVTGDNGDFTLRLEDVSQAQAGTYTCHIHLQEQQLNATVTLAIITVTPKSFGSPGSLGKLLCEVTPVSGQERFVWSSLDTPSQRSFSGPWLEAQEAQLLSQPWQCQLYQGERLLGAAVYFTELSSPGAQRSGRAPGALPAGHLLLFLILGVLSLLLLVTGAFGFHLWRRQWRPRRFSALEQGIHPPQAQSKIEELEQEPEPEPEPEPEPEPEPEPEQL

SEQ ID NO: 39 - protein, 120 aa, Mus musculus
  MISC_FEATURE (1)..(120): Heavy Chain Variable Domain of LAG-3 mAb A
QVQLQQWGAGLLKPSETLSLTCAVYGGSFSDYYWNWIRQPPGKGLEWIGEINHNGNTNSNPSLKSRVTLSLDTSKNQFSLKLRSVTAADTAVYYCAFGYSDYEYNWFDPWGQGTLVTVSS

SEQ ID NO: 40 - protein, 107 aa, Mus musculus
  MISC_FEATURE (1)..(107): Light Chain Variable Domain of LAG-3 mAb A
EIVLTQSPATLSLSPGERATLSCRASQSISSYLAWYQQKPGQAPRLLIYDASNRATGIPARFSGSGSGTDFTLTISSLEPEDFAVYYCQQRSNWPLTFGQGTNLEIK

SEQ ID NO: 41 - protein, 120 aa, Mus musculus
  MISC_FEATURE (1)..(107): Heavy Chain Variable Domain of LAG-3 mAb 1
QIQLVQSGPELKKPGETVKISCKASGYTFRNYGMNWVKQAPGKVLKWMGWINTYTGESTYADDFEGRFAFSLGTSASTAYLQINILKNEDTATYFCARESLYDYYSMDYWGQGTSVTVSS

SEQ ID NO: 42 - protein, 6 aa, Mus musculus
  MISC_FEATURE (1)..(6): CDRH1 of LAG-3 mAb 1
RNYGMN

SEQ ID NO: 43 - protein, 17 aa, Mus musculus
  MISC_FEATURE (1)..(17): CDRH2 of LAG-3 mAb 1
WINTYTGESTYADDFEG

SEQ ID NO: 44 - protein, 11 aa, Mus musculus
  MISC_FEATURE (1)..(11): CDRH3 of LAG-3 mAb 1
ESLYDYYSMDY

SEQ ID NO: 45 - protein, 112 aa, Mus musculus
  MISC_FEATURE (1)..(112): VL Domain of LAG-3 mAb 1
DVVVTQTPLTLSVTIGQPASISCKSSQSLLHSDGKTYLNWLLQRPGQSPERLIYLVSELDSGVPDRFTGSGSGTDFTLKISRVEAEDLGVYYCWQGTHFPYTFGGGTKLEIK

SEQ ID NO: 46 - protein, 16 aa, Mus musculus
  MISC_FEATURE (1)..(16): CDRL1 of LAG-3 mAb 1
KSSQSLLHSDGKTYLN

SEQ ID NO: 47 - protein, 7 aa, Mus musculus
  MISC_FEATURE (1)..(7): CDRL2 of LAG-3 mAb 1
LVSELDS

SEQ ID NO: 48 - protein, 9 aa, Mus musculus
  MISC_FEATURE (1)..(9): CDRL3 of LAG-3 mAb 1
WQGTHFPYT

SEQ ID NO: 49 - protein, 120 aa, Artificial Sequence
  VH Domain of hLAG-3 mAb 1 VH1
QVQLVQSGAEVKKPGASVKVSCKASGYTFTNYGMNWVRQAPGQGLEWMGWINTYTGESTYADDFEGRFVFSMDTSASTAYLQISSLKAEDTAVYYCARESLYDYYSMDYWGQGTTVTVSS

SEQ ID NO: 50 - protein, 120 aa, Artificial Sequence
  VH Domain of hLAG-3 mAb 1 VH2
QVQLVQSGAEVKKPGASVKVSCKASGYTFTNYGMNWVRQAPGQGLEWMGWINTYTGESTYADDFEGRFVFSMDTSASTAYLQISSLKAEDTAVYFCARESLYDYYSMDYWGQGTTVTVSS

SEQ ID NO: 51 - protein, 112 aa, Artificial Sequence
  VH Domain of hLAG-3 mAb 1 VL1
DIVMTQTPLSLSVTPGQPASISCKSSQSLLHSDGKTYLNWLLQKPGQSPERLIYLVSELDSGVPDRFSGSGSGTDFTLKISRVEAEDVGVYYCWQGTHFPYTFGGGTKVEIK

SEQ ID NO: 52 - protein, 112 aa, Artificial Sequence
  VL Domain of hLAG-3 mAb 1 VL2
DIVMTQTPLSLSVTPGQPASISCKSSQSLLHSDGKTYLNWLLQRPGQSPERLIYLVSELDSGVPDRFSGSGSGTDFTLKISRVEAEDVGVYYCWQGTHFPYTFGGGTKVEIK

SEQ ID NO: 53 - protein, 112 aa, Artificial Sequence
  VL Domain of hLAG-3 mAb 1 VL3
DIVMTQTPLSLSVTPGQPASISCKSSQSLLHSDGKTYLNWLLQKPGQPPERLIYLVSELDSGVPDRFSGSGSGTDFTLKISRVEAEDVGVYYCWQGTHFPYTFGGGTKVEIK

SEQ ID NO: 54 - protein, 112 aa, Artificial Sequence
  VL Domain of hLAG-3 mAb 1 VL4
DIVMTQTPLSLSVTPGQPASISCKSSQSLLHSDAKTYLNWLLQKPGQPPERLIYLVSELDSGVPDRFSGSGSGTDFTLKISRVEAEDVGVYYCWQGTHFPYTFGGGTKVEIK

SEQ ID NO: 55 - protein, 16 aa, Artificial Sequence
  CDRL1 of the VL Domain of hLAG-3 mAb 1 VL4
KSSQSLLHSDAKTYLN

SEQ ID NO: 56 - protein, 118 aa, Mus musculus
  MISC_FEATURE (1)..(118): VH Domain of LAG-3 mAb 6
EVLLQQSGPELVKPGASVKIPCKASGYTFTDYNMDWVKQSHGESLEWIGDINPDNGVTIYNQKFEGKATLTVDKSSSTAYMELRSLTSEDTAVYYCAREADYFYFDYWGQGTTLTVSS

SEQ ID NO: 57 - protein, 5 aa, Mus musculus
  MISC_FEATURE (1)..(5): CDRH1 of LAG-3 mAb 6
DYNMD

SEQ ID NO: 58 - protein, 17 aa, Mus musculus
  MISC_FEATURE (1)..(17): CDRH2 of LAG-3 mAb 6
DINPDNGVTIYNQKFEG

SEQ ID NO: 59 - protein, 9 aa, Mus musculus
  MISC_FEATURE (1)..(9): CDRH3 of LAG-3 mAb 6
EADYFYFDY

SEQ ID NO: 60 - protein, 107 aa, Mus musculus
  MISC_FEATURE (1)..(107): VL Domain of LAG-3 mAb 6
DIVMTQSHRFMSTSVGDRVSITCKASQDVSSVVAWYQQKPGQSPKLLIFSASYRYTGVPDRFTGSGSGTDFTFTISSVQAADLAVYYCQQHYSTPWTFGGGTKLEIK

SEQ ID NO: 61 - protein, 11 aa, Mus musculus
  MISC_FEATURE (1)..(11): CDRL1 of LAG-3 mAb 6
KASQDVSSVVA

SEQ ID NO: 62 - protein, 7 aa, Mus musculus
  MISC_FEATURE (1)..(7): CDRL2 of LAG-3 mAb 6
SASYRYT

SEQ ID NO: 63 - protein, 7 aa, Mus musculus
  MISC_FEATURE (1)..(7): CDRL3 of LAG-3 mAb 6
HYSTPWT

SEQ ID NO: 64 - protein, 113 aa, Homo sapiens [sequence omitted]

SEQ ID NO: 65 - protein, 107 aa, Homo sapiens [sequence omitted]

SEQ ID NO: 66 - protein, 120 aa, Homo sapiens [sequence omitted]

SEQ ID NO: 67 - protein, 111 aa, Homo sapiens [sequence omitted]

SEQ ID NO: 68 - protein, 288 aa, Homo sapiens
  MISC_FEATURE (1)..(288): Human PD-1 Polypeptide (NCI Sequence NP 005009.2)
  MISC_FEATURE (1)..(20): Human PD-1 Signal Sequence
MQIPQAPWPVVWAVLQLGWRPGWFLDSPDRPWNPPTFSPALLVVTEGDNATFTCSFSNTSESFVLNWYRMSPSNQTDKLAAFPEDRSQPGQDCRFRVTQLPNGRDFHMSVVRARRNDSGTYLCGAISLAPKAQIKESLRAELRVTERRAEVPTAHPSPSPRPAGQFQTLVVGVVGGLLGSLVLLVWVLAVICSRAARGTIGARRTGQPLKEDPSAVPVFSVDYGELDFQWREKTPEPPVPCVPEQTEYATIVFPSGMGTSSPARRGSADGPRSAQPLRPEDGHCSWPL

SEQ ID NO: 69 - protein, 121 aa, Mus musculus
  MISC_FEATURE (1)..(121): VH Domain of PD-1 mAb 1
DVQLQESGPGRVKPSQSLSLTCTVTGFSITNDYAWNWIRQFPGNKLEWMGHITYSGSTSYNPSLKSRISITRDTSKNHFFLQLSSVTPEDTATYYCARDYGSGYPYTLDYWGQGTSVTVSS

SEQ ID NO: 70 - DNA, 373 bp, Mus musculus
  misc_feature (1)..(373): Polynucleotide Encoding VH Domain of PD-1 mAb 1
cagatccagtgatgtgcagcttcaggagtcgggacctggccgggtgaaaccttctcagtctctgtccctcacctgcactgtcactggcttctcaatcaccaatgattatgcctggaactggatccgacagtttccaggaaacaaactggagtggatgggccacataacctacagtggcagcactagctacaacccatctctcaaaagtcgaatctctatcactcgggacacatccaagaaccacttcttcctgcagttgagttctgtgactcctgaggacacagccacatattactgtgcaagagattacggtagtggctacccctatactttggactactggggtcaaggtacctcagtcaccgtctcctcc

SEQ ID NO: 71 - protein, 6 aa, Mus musculus
  MISC_FEATURE (1)..(6)
NDYAWN

SEQ ID NO: 72 - protein, 16 aa, Mus musculus
  MISC_FEATURE (1)..(16): CDRH2 of PD-1 mAb 1
HITYSGSTSYNPSLKS

SEQ ID NO: 73 - protein, 12 aa, Mus musculus
  MISC_FEATURE (1)..(12): CDRH3 of PD-1 mAb 1
DYGSGYPYTLDY

SEQ ID NO: 74 - protein, 106 aa, Mus musculus
  MISC_FEATURE (1)..(106): VL Domain of PD-1 mAb 1
QIVLTQSPALMSASPGEKVTMTCSATSIVSYVYWYQQKPGSSPQPWIYLTSNLASGVPARFSGSGSGTSYSLTISSMEAEDAATYYCQQWSDNPYTFGGGTKLEIK

SEQ ID NO: 75 - DNA, 318 bp, Mus musculus
  misc_feature (1)..(318): Polynucleotide Encoding VL Domain of PD-1 mAb 1
caaattgttctcacccagtctccagcactcatgtctgcatctccaggggagaaggtcaccatgacctgcagtgccacctcaattgtaagttacgtttactggtaccagcagaagcctggatcctccccccaaccctggatttatctcacatccaacctggcttctggagtccctgctcgcttcagtggcagtgggtctgggacctcttactctctcacaatcagcagcatggaggctgaagatgctgccacttattactgccagcagtggagtgataacccgtacacgttcggaggggggaccaagctggaaataaaa

SEQ ID NO: 76 - protein, 10 aa, Mus musculus
  MISC_FEATURE (1)..(10): CDRL1 of PD-1 mAb 1
SATSIVSYVY

SEQ ID NO: 77 - protein, 7 aa, Mus musculus
  MISC_FEATURE (1)..(7): CDRL2 of PD-1 mAb 1
LTSNLAS

SEQ ID NO: 78 - protein, 9 aa, Mus musculus
  MISC_FEATURE (1)..(9): CDRL3 of PD-1 mAb 1
QQWSDNPYT

SEQ ID NO: 79 - protein, 121 aa, Artificial Sequence
  VH Domain of hPD-1 mAb 1 VH1
DVQLQESGPGLVKPSQTLSLTCTVSGFSISNDYAWNWIRQPPGKGLEWIGHITYSGSTSYNPSLKSRLTITRDTSKNQFVLTMTNMDPVDTATYYCARDYGSGYPYTLDYWGQGTTVTVSS

SEQ ID NO: 80 - DNA, 363 bp, Artificial Sequence
  Polynucleotide Encoding hPD-1 mAb 1 VH1
gacgtacagctccaggaaagtggcccaggtctggtgaagccatcccagacactgagcctgacttgcaccgtgagtggcttctccatctcaaatgactacgcctggaattggattaggcagcctcccggtaaagggctggagtggatcggccacatcacatacagcggctccacatcatataatcccagtctgaagagccgtcttaccattactcgcgacactagtaagaaccagtttgttctgaccatgaccaacatggaccctgtggatactgcaacatactattgtgctcgagattatggttctggttacccttatacactcgactactggggacagggaaccactgtgaccgtgagctcc

SEQ ID NO: 81 - protein, 106 aa, Artificial Sequence
  VL Domain of hPD-1 mAb 1 VL1
EIVLTQSPATLSVSPGEKVTITCSATSIVSYVYWYQQKPGQAPQPLIYLTSNLASGIPARFSGSGSGTDFTLTISSLEAEDAATYYCQQWSDNPYTFGGGTKVEIK

SEQ ID NO: 82 - DNA, 318 bp, Artificial Sequence
  Polynucleotide Encoding hPD-1 mAb 1 VL1
gaaatcgttctgacccagagcccagcaaccctgtctgtctcccccggagaaaaggtcaccattacttgctctgctacttctatcgtgtcctacgtgtactggtatcagcagaagcccggtcaggctccccagccattgatatatctgaccagcaacctggcttctggtatcccagctcgtttttccggtagcgggtccgggactgatttcactttgactatcagctctctggaggcagaagacgccgccacctattattgtcaacagtggtcagacaatccatacacttttggcggtggcaccaaagtcgaaataaag

SEQ ID NO: 83 - protein, 116 aa, Mus musculus
  MISC_FEATURE (1)..(116): VH Domain of PD-1 mAb 2
DVQLVESGGGLVQPGGSRKLSCAASGFVFSSFGMHWVRQAPEKGLEWVAYISSGSMSISYADTVKGRFTVTRDNAKNTLFLQMTSLRSEDTAIYYCASLSDYFDYWGQGTTLTVSS

SEQ ID NO: 84 - DNA, 348 bp, Mus musculus
  misc_feature (1)..(348): Polynucleotide Encoding the VH Domain of PD-1 mAb 2
gatgtgcagctcgtggagtctgggggaggcttagtgcagcctggagggtcccggaaactctcctgtgcagcctctggattcgttttcagtagctttggaatgcactgggttcgtcaggctccagagaaggggctggagtgggtcgcatacatcagtagtggcagtatgagcatttcctatgcagacacagtgaagggccgattcaccgtcaccagagacaatgccaagaacaccctgttcctgcaaatgaccagtctaaggtctgaggacacggccatttattactgtgcatccctgagtgactactttgactactggggccaaggcaccactctcacagtctcctcc

SEQ ID NO: 85 - protein, 5 aa, Mus musculus
  MISC_FEATURE (1)..(5): CDRH1 of PD-1 mAb 2
SFGMH

SEQ ID NO: 86 - protein, 17 aa, Mus musculus
  MISC_FEATURE (1)..(17): CDRH2 of PD-1 mAb 2
YISSGSMSISYADTVKG

SEQ ID NO: 87 - protein, 7 aa, Mus musculus
  MISC_FEATURE (1)..(7): CDRH3 of PD-1 mAb 2
LSDYFDY

SEQ ID NO: 88 - protein, 112 aa, Mus musculus
  MISC_FEATURE (1)..(112): VL Domain of PD-1 mAb 2
DVVMSQTPLSLPVSLGDQASISCRSSQSLVHSTGNTYLHWYLQKPGQSPKLLIYRVSNRFSGVPDRFSGSGSGTDFTLKISRVEAEDLGVFFCSQTTHVPWTFGGGTKLEIK

SEQ ID NO: 89 - DNA, 336 bp, Mus musculus
  misc_feature (1)..(336): Polynucleotide Encoding the VL Domain of PD-1 mAb 2
gatgttgtgatgtcccaaactccactctccctgcctgtcagtcttggagatcaagcctccatctcttgcagatctagtcagagccttgttcacagtactggaaacacctatttacattggtacctgcagaagccaggccagtctccaaagctcctgatctacagggtttctaaccgattttctggggtccccgacaggttcagtggcagtggatcagggacagatttcacactcaagatcagtagagtggaggctgaggatctgggagtttttttctgctctcaaactacacatgttccgtggacgttcggtggaggcaccaagctggaaatcaaa

SEQ ID NO: 90 - protein, 16 aa, Mus musculus
  MISC_FEATURE (1)..(16): CDRL1 of PD-1 mAb 2
RSSQSLVHSTGNTYLH

SEQ ID NO: 91 - protein, 7 aa, Mus musculus
  MISC_FEATURE (1)..(7): CDRL2 of PD-1 mAb 2
RVSNRFS

SEQ ID NO: 92 - protein, 9 aa, Mus musculus
  MISC_FEATURE (1)..(9): CDRL3 of PD-1 mAb 2
SQTTHVPWT

SEQ ID NO: 93 - protein, 116 aa, Artificial Sequence
  VH Domain of hPD-1 mAb 2 VH1
EVQLVESGGGLVQPGGSLRLSCAASGFVFSSFGMHWVRQAPGKGLEWVAYISSGSMSISYADTVKGRFTISRDNAKNTLYLQMNSLRTEDTALYYCASLSDYFDYWGQGTTVTVSS

SEQ ID NO: 94 - DNA, 348 bp, Artificial Sequence
  Polynucleotide Encoding hPD-1 mAb 2 VH1
gaagtgcaattggttgagagtggtggtggcctggtgcagccaggtggaagtctgcggttgtcctgtgcagcaagcggatttgtgttcagctcttttgggatgcattgggtgcgccaggctcccggcaagggtctcgagtgggtagcatacatctccagcgggtccatgtctattagttatgccgacacagtgaaaggcaggtttactatctcccgtgacaatgcaaaaaacacactgtacctgcaaatgaatagcctgcgcaccgaggacaccgccttgtactactgcgcttccctgtctgattacttcgactactggggtcagggcacaactgtgacagtttcttcc

SEQ ID NO: 95 - protein, 112 aa, Artificial Sequence
  VL Domain of hPD-1 mAb 2 VL1
DVVMTQSPLSLPVTLGQPASISCRSSQSLVHSTGNTYLHWYLQKPGQSPQLLIYRVSNRFSGVPDRFSGSGSGTDFTLKISRVEAEDVGVYYCSQTTHVPWTFGQGTKLEIK

SEQ ID NO: 96 - DNA, 336 bp, Artificial Sequence
  Polynucleotide Encoding hPD-1 mAb 2 VL1
gacgttgtgatgacacagtcaccactgagtctgccagttaccctgggccagccagccagtatttcttgtcggagttcacagagtctggtacattccacaggaaatacatatctccattggtacctgcaaaaaccagggcagagcccccagctgctgatttatagagtgtctaatcgattttctggcgtgccagatcggttcagcggcagcgggtctggcactgatttcacactgaaaatctctagggtggaggcagaggacgtaggcgtttactactgtagtcagaccacccatgtaccctggacttttggccaaggtactaagctggaaatcaag

SEQ ID NO: 97 - protein, 125 aa, Mus musculus
  MISC_FEATURE (1)..(125): VH Domain of PD-1 mAb 3
QVQLQQSGAELVRPGASVTLSCKASGYTFTDYVMHWVKQTPVHGLEWIGTIDPETGGTAYNQKFKGKAILTADKSSNTAYMELRSLTSEDSAVYYFTREKITTIVEGTYWYFDVWGTGTTVTVSS

SEQ ID NO: 98 - DNA, 375 bp, Mus musculus
  misc_feature (1)..(375): Polynucleotide Encoding the VH Domain of PD-1 mAb 3
caggttcaactgcaacagtctggggctgagctggtgaggcctggggcttcagtgacgctgtcctgcaaggcttcgggctacacatttactgactatgtaatgcactgggtgaagcagacacctgtgcatggcctggaatggattggaactattgatcctgaaactggtggtactgcctacaatcagaagttcaagggcaaggccatactgactgcagacaagtcctccaacacagcctacatggagctccgcagcctgacatctgaggactctgccgtctattactttacaagagagaagattactacgatagtagaggggacatactggtacttcgatgtctggggcacagggaccacggtcaccgtctcctca

SEQ ID NO: 99 - protein, 5 aa, Mus musculus
  MISC_FEATURE (1)..(5): CDRH1 of PD-1 mAb 3
DYVMH

SEQ ID NO: 100 - protein, 17 aa, Mus musculus
  MISC_FEATURE (1)..(17): CDRH2 of PD-1 mAb 3
TIDPETGGTAYNQKFKG

SEQ ID NO: 101 - protein, 16 aa, Mus musculus
  MISC_FEATURE (1)..(16): CDRH3 of PD-1 mAb 3
EKITTIVEGTYWYFDV

SEQ ID NO: 102 - protein, 112 aa, Mus musculus
  MISC_FEATURE (1)..(112): VL Domain of PD-1 mAb 3
DVLLTQTPLSLPVSLGDQASISCRSSQNIVHSNGDTYLEWYLQKPGQSPKLLIYKVSNRFSGVPDRFSGSGSGTDFTLKISRVEAEDLGVYYCFQGSHLPYTFGGGTKLEIK

SEQ ID NO: 103 - DNA, 336 bp, Mus musculus
  misc_feature (1)..(336): Polynucleotide Encoding the VL Domain of PD-1 mAb 3
gatgttttgctgacccaaactccactctccctgcctgtcagtcttggagatcaagcctccatctcttgcagatctagtcagaacattgtacatagtaatggagacacctatttggaatggtacctgcagaaaccaggccagtctccaaagctcctgatctataaagtttccaaccgattttctggggtcccagacaggttcagtggcagtgggtcagggacagattttacactcaaaatcagcagagtggaggctgaggatctgggagtttattactgctttcaaggttcacatcttccgtacacgttcggaggggggaccaagctggaaataaaa

SEQ ID NO: 104 - protein, 16 aa, Mus musculus
  MISC_FEATURE (1)..(16): CDRL1 of PD-1 mAb 3
RSSQNIVHSNGDTYLE

SEQ ID NO: 105 - protein, 7 aa, Mus musculus
  MISC_FEATURE (1)..(7): CDRL2 of PD-1 mAb 3
KVSNRFS

SEQ ID NO: 106 - protein, 9 aa, Mus musculus
  MISC_FEATURE (1)..(9): CDRL3 of PD-1 mAb 3
FQGSHLPYT

SEQ ID NO: 107 - protein, 116 aa, Mus musculus
  MISC_FEATURE (1)..(116): VH Domain of PD-1 mAb 4
DVQLVESGGGLVQPGGSRKLSCAASGFVFSSFGMHWVRQAPEKGLEWVAYISSGSMSISYADTVKGRFTVTRDNAKNTLFLQMTSLRSEDTAIYYCASLTDYFDYWGQGTTLTVSS

SEQ ID NO: 108 - DNA, 348 bp, Mus musculus
  misc_feature (1)..(348): Polynucleotide Encoding the VH Domain of PD-1 mAb 4
gatgtgcagctcgtggagtctgggggaggcttagtgcagcctggagggtcccggaaactctcctgtgcagcctctggattcgttttcagtagctttggaatgcactgggttcgtcaggctccagagaaggggctggagtgggtcgcatatattagtagtggcagtatgagtatttcctatgcagacacagtgaagggccgattcaccgtcaccagagacaatgccaagaacaccctgttcctgcaaatgaccagtctaaggtctgaggacacggccatttattactgtgcatccctgactgactactttgactactggggccaaggcaccactctcacagtctcctca

SEQ ID NO: 109 - protein, 5 aa, Mus musculus
  MISC_FEATURE (1)..(5): CDRH1 of PD-1 mAb 4
SFGMH

SEQ ID NO: 110 - protein, 17 aa, Mus musculus
  MISC_FEATURE (1)..(17): CDRH2 of PD-1 mAb 4
YISSGSMSISYADTVKG

SEQ ID NO: 111 - protein, 7 aa, Mus musculus
  MISC_FEATURE (1)..(7): CDRH3 of PD-1 mAb 4
LTDYFDY

SEQ ID NO: 112 - protein, 112 aa, Mus musculus
  MISC_FEATURE (1)..(112): VL Domain of PD-1 mAb 4
DVVMSQTPLSLPVSLGDQASISCRSSQSLVHSTGNTYFHWYLQKPGQSPKLLIYRVSNRFSGVPDRFSGSGSGTDFTLKISRVEAEDLGVYFCSQTTHVPWTFGGGTKLEIK

SEQ ID NO: 113 - DNA, 336 bp, Mus musculus
  misc_feature (1)..(336): Polynucleotide Encoding the VL Domain of PD-1 mAb
gatgttgtgatgtcccaaactccactctccctgcctgtcagtcttggagatcaagcctccatctcctgcagatctagtcagagccttgttcacagtactggaaacacctatttccattggtacctgcagaagccaggccagtctccaaagctcctgatctacagggtttctaaccgattttctggggtccccgacaggttcagtggcagtggatcagggacagatttcacactcaagatcagcagagtggaggctgaggatctgggagtttatttctgctctcaaactacacatgttccgtggacgttcggtggaggcaccaagctggaaatcaaa

SEQ ID NO: 114 - protein, 16 aa, Mus musculus
  MISC_FEATURE (1)..(16): CDRL1 of PD-1 mAb 4
RSSQSLVHSTGNTYFH

SEQ ID NO: 115 - protein, 7 aa, Mus musculus
  MISC_FEATURE (1)..(7): CDRL2 of PD-1 mAb 4
RVSNRFS

SEQ ID NO: 116 - protein, 9 aa, Mus musculus
  MISC_FEATURE (1)..(9): CDRL3 of PD-1 mAb 4
SQTTHVPWT

SEQ ID NO: 117 - protein, 119 aa, Mus musculus
  MISC_FEATURE (1)..(119): VH Domain of PD-1 mAb 5
QVQLQQPGVELVRPGASVKLSCKASGYSFTAYWMNWMKQRPGQGLEWIGVIHPSDSETWLNQKFKDKATLTVDKSSSTAYMQLISPTSEDSAVYYCAREHYGSSPFAYWGQGTLVTVSA

SEQ ID NO: 118 - DNA, 357 bp, Mus musculus
  misc_feature (1)..(357): Polynucleotide Encoding the VH Domain of PD-1 mAb 5
caggtccaactgcagcagcctggggttgaactggtgaggcctggagcttcagtgaagctgtcctgcaaggcttctggctactccttcaccgcctactggatgaactggatgaaacagaggcctggacaaggccttgagtggattggcgtgattcatccttccgatagtgaaacttggttaaatcagaagttcaaggacaaggccacattgactgtagacaaatcctccagcacagcctacatgcaactcatcagcccgacatctgaggactctgcggtctattactgtgcaagagagcactacggtagtagcccgtttgcttactggggccaagggactctggtcactgtctctgca

SEQ ID NO: 119 - protein, 5 aa, Mus musculus
  MISC_FEATURE (1)..(5): CDRH1 of PD-1 mAb 5
AYWMN

SEQ ID NO: 120 - protein, 17 aa, Mus musculus
  MISC_FEATURE (1)..(17): CDRH2 of PD-1 mAb 5
VIHPSDSETWLNQKFKD

SEQ ID NO: 121 - protein, 10 aa, Mus musculus
  MISC_FEATURE (1)..(10): CDRH3 of PD-1 mAb 5
EHYGSSPFAY

SEQ ID NO: 122 - protein, 111 aa, Mus musculus
  MISC_FEATURE (1)..(111): VL Domain of PD-1 mAb 5
DIVLTQSPASLAVSLGQRATISCRANESVDNYGMSFMNWFQQKPGQPPKLLIYAASNQGSGVPARFSGSGSGTDFSLNIHPMEEDDTAMYFCQQSKEVPYTFGGGTKLEIK

SEQ ID NO: 123 - DNA, 333 bp, Mus musculus
  misc_feature (1)..(333): Polynucleotide Encoding the VL Domain of PD-1 mAb 5
gacattgtgctgacccaatctccagcttctttggctgtgtctctagggcagagggccaccatctcctgcagagccaacgaaagtgttgataattatggcatgagttttatgaactggttccaacagaaaccaggacagccacccaaactcctcatctatgctgcatccaaccaaggatccggggtccctgccaggtttagtggcagtgggtctgggacagatttcagcctcaacatccatcctatggaggaggatgatactgcaatgtatttctgtcagcaaagtaaggaggttccgtacacgttcggaggggggaccaagctggaaataaaa

SEQ ID NO: 124 - protein, 15 aa, Mus musculus
  MISC_FEATURE (1)..(15): CDRL1 of PD-1 mAb 5
RANESVDNYGMSFMN

SEQ ID NO: 125 - protein, 7 aa, Mus musculus
  MISC_FEATURE (1)..(7): CDRL2 of PD-1 mAb 5
AASNQGS

SEQ ID NO: 126 - protein, 9 aa, Mus musculus
  MISC_FEATURE (1)..(9): CDRL3 of PD-1 mAb 5
QQSKEVPYT

SEQ ID NO: 127 - protein, 118 aa, Mus musculus
  MISC_FEATURE (1)..(118): VH Domain of PD-1 mAb 6
EVKLVESGGGLVNPGGSLKLSCAASGFTFSSYGMSWVRQTPEKRLEWVATISGGGSDTYYPDSVKGRFTISRDNAKNNLYLQMSSLRSEDTALYYCARQKATTWFAYWGQGTLVTVST

SEQ ID NO: 128 - DNA, 333 bp, Mus musculus
  misc_feature (1)..(333): Polynucleotide Encoding the VH Domain of PD-1 mAb 6
gaaatcgtactcacccagtcacctgcaaccctttctctgagccccggtgaacgtgccactctcagctgcagagcaagtgagagtgtggacaattacggcatgtccttcatgaactggtttcagcagaagcctgggcagccacctaagctgctcatccacgccgcctctaaccgcggatctggggtgccttcacgtttttctggatcaggaagtggcactgacttcacccttacaatcagctctctggagccagaggactttgccgtctatttctgccagcaatctaaagaggtgccctatacttttggtggcgggaccaaggttgagatcaaa

SEQ ID NO: 129 - protein, 5 aa, Mus musculus
  MISC_FEATURE (1)..(5): CDRH1 of PD-1 mAb 6
SYGMS

SEQ ID NO: 130 - protein, 17 aa, Mus musculus
  MISC_FEATURE (1)..(17): CDRH2 of PD-1 mAb 6
TISGGGSDTYYPDSVKG

SEQ ID NO: 131 - protein, 9 aa, Mus musculus
  MISC_FEATURE (1)..(9): CDRH3 of PD-1 mAb 6
QKATTWFAY

SEQ ID NO: 132 - protein, 111 aa, Mus musculus
  MISC_FEATURE (1)..(111): VL Domain of PD-1 mAb 6
DIVLTQSPASLAVSLGQRATISCRASESVDNYGISFMNWFQQKPGQPPKLLIYPASNQGSGVPARFSGSGSGTDFSLNIHPMEEDDAAMYFCQQSKEVPWTFGGGTKLEIK

SEQ ID NO: 133 - DNA, 333 bp, Mus musculus
  misc_feature (1)..(333): Polynucleotide Encoding the VL Domain of PD-1 mAb 6
gacattgtgctgacccaatctccagcttctttggctgtgtctctagggcagagggccaccatctcctgcagagccagcgaaagtgttgataattatggcattagttttatgaactggttccaacagaaaccaggacagccacccaaactcctcatctatcctgcatccaaccaaggatccggggtccctgccaggtttagtggcagtgggtctgggacagacttcagcctcaacatccatcctatggaggaggatgatgctgcaatgtatttctgtcagcaaagtaaggaggttccgtggacgttcggtggaggcaccaagctggaaatcaaa

SEQ ID NO: 134 - protein, 15 aa, Mus musculus
  MISC_FEATURE (1)..(15): CDRL1 of PD-1 mAb 6
RASESVDNYGISFMN

SEQ ID NO: 135 - protein, 7 aa, Mus musculus
  MISC_FEATURE (1)..(7): CDRL2 of PD-1 mAb 6
PASNQGS

SEQ ID NO: 136 - protein, 9 aa, Mus musculus
  MISC_FEATURE (1)..(9): CDRL3 of PD-1 mAb 6
QQSKEVPWT

SEQ ID NO: 137 - protein, 119 aa, Mus musculus
  MISC_FEATURE (1)..(119): VH Domain of PD-1 mAb 7
QVQLQQPGAELVRPGASVKLSCKASGYSFTSYWMNWVKQRPGQGLEWIGVIHPSDSETWLDQKFKDKATLTVDKSSTTAYMQLISPTSEDSAVYYCAREHYGTSPFAYWGQGTLVTVSS

SEQ ID NO: 138 - DNA, 357 bp, Mus musculus
  misc_feature (1)..(357): Polynucleotide Encoding the VH Domain of PD-1 mAb 7
gaggtccaactgcagcagcctggggctgaactggtgaggcctggagcttcagtgaagctgtcctgcaaggcttctggctactccttcaccagctactggatgaactgggtgaagcagaggcctggacaaggccttgagtggattggcgtgattcatccttccgatagtgaaacttggttagatcagaagttcaaggacaaggccacattgactgtagacaaatcctccaccacagcctacatgcaactcatcagcccgacatctgaggactctgcggtctattactgtgcaagggagcactacggtactagcccgtttgcttactggggccaagggactctggtcactgtgtcttcc

SEQ ID NO: 139 - protein, 5 aa, Mus musculus
  MISC_FEATURE (1)..(5): CDRH1 of PD-1 mAb 7
SYWMN

SEQ ID NO: 140 - protein, 17 aa, Mus musculus
  MISC_FEATURE (1)..(17): CDRH2 of PD-1 mAb 7
VIHPSDSETWLDQKFKD

SEQ ID NO: 141 - protein, 10 aa, Mus musculus
  MISC_FEATURE (1)..(10): CDRH3 of PD-1 mAb 7
EHYGTSPFAY

SEQ ID NO: 142 - protein, 111 aa, Mus musculus
  MISC_FEATURE (1)..(111): VL Domain of PD-1 mAb 7
DIVLTQSPASLAVSLGQRATISCRANESVDNYGMSFMNWFQQKPGQPPKLLIHAASNQGSGVPARFSGSGFGTDFSLNIHPMEEDDAAMYFCQQSKEVPYTFGGGTKLEIK

SEQ ID NO: 143 - DNA, 333 bp, Mus musculus
  misc_feature (1)..(333): Polynucleotide Encoding the VL Domain of PD-1 mAb 7
gacattgtgctgacccaatctccagcttctttggctgtgtctctagggcagagggccaccatctcctgcagagccaacgaaagtgttgataattatggcatgagttttatgaactggttccaacagaaaccaggacagccacccaaactcctcatccatgctgcatccaaccaaggatccggggtccctgccaggtttagtggcagtgggtttgggacagacttcagcctcaacatccatcctatggaggaggatgatgctgcaatgtatttctgtcagcaaagtaaggaggttccgtacacgttcggaggggggaccaagctggaaataaaa

SEQ ID NO: 144 - protein, 15 aa, Mus musculus
  MISC_FEATURE (1)..(15): CDRL1 of PD-1 mAb 7
RANESVDNYGMSFMN

SEQ ID NO: 145 - protein, 7 aa, Mus musculus
  MISC_FEATURE (1)..(7): CDRL2 of PD-1 mAb 7
AASNQGS

SEQ ID NO: 146 - protein, 9 aa, Mus musculus
  MISC_FEATURE (1)..(9): CDRL3 of PD-1 mAb 7
QQSKEVPYT

SEQ ID NO: 147 - protein, 119 aa, Artificial Sequence
  VH Domain of hPD-1 mAb 7 VH1
QVQLVQSGAEVKKPGASVKVSCKASGYSFTSYWMNWVRQAPGQGLEWIGVIHPSDSETWLDQKFKDRVTITVDKSTSTAYMELSSLRSEDTAVYYCAREHYGTSPFAYWGQGTLVTVSS

SEQ ID NO: 148 - DNA, 357 bp, Artificial Sequence
  Polynucleotide Encoding hPD-1 mAb 7 VH1
caagttcaattggtacagagcggggcagaggtgaagaaacccggcgccagtgttaaggtgtcctgcaaagccagcggttacagctttacaagctattggatgaattgggtgcgtcaagcaccagggcagggtctggaatggattggggtgatacatccttctgacagcgaaacatggttggaccagaaatttaaagatcgtgtgacaattacagtcgataagtccacaagcactgcttacatggaactctccagcttgcggtccgaggacaccgctgtgtattattgcgccagagagcactacggcacatcaccttttgcatactggggccagggaactctcgtaaccgtatcctcc

SEQ ID NO: 149 - protein, 119 aa, Artificial Sequence
  VH Domain of hPD-1 mAb 7 VH2
QVQLVQSGAEVKKPGASVKVSCKASGYSFTSYWMNWVRQAPGQGLEWAGVIHPSDSETWLDQKFKDRVTITVDKSTSTAYMELSSLRSEDTAVYYCAREHYGTSPFAYWGQGTLVTVSS

SEQ ID NO: 150 - DNA, 357 bp, Artificial Sequence
  Polynucleotide Encoding hPD-1 mAb 7 VH2
caagttcaattggtacagagcggggcagaggtgaagaaacccggcgccagtgttaaggtgtcctgcaaagccagcggttacagctttacaagctattggatgaattgggtgcgtcaagcaccagggcagggtctggaatgggctggggtgatacatccttctgacagcgaaacatggttggaccagaaatttaaagatcgtgtgacaattacagtcgataagtccacaagcactgcttacatggaactctccagcttgcggtccgaggacaccgctgtgtattattgcgccagagagcactacggcacatcaccttttgcatactggggccagggaactctcgtaaccgtatcctcc

SEQ ID NO: 151 - protein, 111 aa, Artificial Sequence
  VL Domain of hPD-1 mAb 7 VL1
EIVLTQSPATLSLSPGERATLSCRANESVDNYGMSFMNWFQQKPGQPPKLLIHAASNQGSGVPSRFSGSGSGTDFTLTISSLEPEDFAVYFCQQSKEVPYTFGGGTKVEIK

SEQ ID NO: 152 - DNA, 333 bp, Artificial Sequence
  Polynucleotide Encoding hPD-1 mAb 7 VL1
gaaatcgtactcacccagtcacctgcaaccctttctctgagccccggtgaacgtgccactctcagctgcagagcaaatgagagtgtggacaattacggcatgtccttcatgaactggtttcagcagaagcctgggcagccacctaagctgctcatccacgccgcctctaaccagggatctggggtgccttcacgtttttctggatcaggaagtggcactgacttcacccttacaatcagctctctggagccagaggactttgccgtctatttctgccagcaatctaaagaggtgccctatacttttggtggcgggaccaaggttgagatcaaa

SEQ ID NO: 153 - protein, 111 aa, Artificial Sequence
  VL Domain of hPD-1 mAb 7 VL2
EIVLTQSPATLSLSPGERATLSCRASESVDNYGMSFMNWFQQKPGQPPKLLIHAASNQGSGVPSRFSGSGSGTDFTLTISSLEPEDFAVYFCQQSKEVPYTFGGGTKVEIK

SEQ ID NO: 154 - DNA, 333 bp, Artificial Sequence
  Polynucleotide Encoding hPD-1 mAb 7 VL2
gaaatcgtactcacccagtcacctgcaaccctttctctgagccccggtgaacgtgccactctcagctgcagagcaagtgagagtgtggacaattacggcatgtccttcatgaactggtttcagcagaagcctgggcagccacctaagctgctcatccacgccgcctctaaccagggatctggggtgccttcacgtttttctggatcaggaagtggcactgacttcacccttacaatcagctctctggagccagaggactttgccgtctatttctgccagcaatctaaagaggtgccctatacttttggtggcgggaccaaggttgagatcaaa

SEQ ID NO: 155 - protein, 111 aa, Artificial Sequence
  VL Domain of hPD-1 mAb 7 VL3
EIVLTQSPATLSLSPGERATLSCRASESVDNYGMSFMNWFQQKPGQPPKLLIHAASNRGSGVPSRFSGSGSGTDFTLTISSLEPEDFAVYFCQQSKEVPYTFGGGTKVEIK

SEQ ID NO: 156 - DNA, 333 bp, Artificial Sequence; identical to SEQ ID NO: 128
  Polynucleotide Encoding hPD-1 mAb 7 VL3

SEQ ID NO: 157 - protein, 15 aa, Artificial Sequence
  CDRL1 of the VL Domain of hPD-1 mAb 7 VL2 and hPD-1 mAb 7 VL3
RASESVDNYGMSFMN

SEQ ID NO: 158 - protein, 7 aa, Artificial Sequence
  CDRL2 of the VL Domain of hPD-1 mAb 7 VL3
AASNRGS

SEQ ID NO: 159 - protein, 113 aa, Mus musculus
  MISC_FEATURE (1)..(113): VH Domain of PD-1 mAb 8
EGQLQQSGPELVKPGASVKISCKASGYTFTDYYMNWVKQNHGKSLEWIGDINPKNGDTHYNQKFKGEATLTVDKSSTTAYMELRSLTSEDSAVYYCASDFDYWGQGTTLTVSS

SEQ ID NO: 160 - DNA, 339 bp, Mus musculus
  misc_feature (1)..(339): Polynucleotide Encoding the VH Domain of PD-1 mAb 8
gagggccagctgcaacaatctggacctgagctggtgaagcctggggcttcagtgaagatatcctgtaaggcttctggatacacgttcactgactactacatgaactgggtgaagcagaaccatggaaagagccttgagtggattggagatattaatcctaaaaatggtgacactcactacaaccagaagttcaagggcgaggccacattgactgtagacaagtcctccaccacagcctacatggagctccgcagcctgacatctgaggactctgcagtctattactgtgcgagcgattttgactactggggccaaggcaccactctcacagtctcctcc

SEQ ID NO: 161 - protein, 5 aa, Mus musculus
  MISC_FEATURE (1)..(5): CDRH1 of PD-1 mAb 8
DYYMN

SEQ ID NO: 162 - protein, 17 aa, Mus musculus
  MISC_FEATURE (1)..(17): CDRH2 of PD-1 mAb 8
DINPKNGDTHYNQKFKG

SEQ ID NO: 163 - protein, 4 aa, Mus musculus
  MISC_FEATURE (1)..(4): CDRH3 of PD-1 mAb 8
DFDY

SEQ ID NO: 164 - protein, 112 aa, Mus musculus
  MISC_FEATURE (1)..(112): VL Domain of PD-1 mAb 8
DVVMTQTPLSLPVGLGDQASISCRSSQTLVYSNGNTYLNWFLQKPGQSPKLLIYKVSNRFSGVPDRFSGSGSGTDFTLKISRVEAEDLGVYFCSQSTHVPFTFGSGTKLEIK

SEQ ID NO: 165 - DNA, 336 bp, Mus musculus
  misc_feature (1)..(336): Polynucleotide Encoding the VL Domain of PD-1 mAb 8
gatgttgtgatgacccaaactccactctccctgcctgtcggtcttggagatcaagcctccatctcttgcagatctagtcagacccttgtatatagtaatggaaacacctatttaaattggttcctgcagaagccaggccagtctccaaagctcctgatctacaaagtttccaaccgattttctggggtcccagacaggttcagtggcagtggatcagggacagatttcacactcaagatcagcagagtggaggctgaggatctgggagtttatttctgctctcaaagtacacatgttccattcacgttcggctcggggacaaagttggaaataaaa

SEQ ID NO: 166 - protein, 16 aa, Mus musculus
  MISC_FEATURE (1)..(16): CDRL1 of PD-1 mAb 8
RSSQTLVYSNGNTYLN

SEQ ID NO: 167 - protein, 7 aa, Mus musculus
  MISC_FEATURE (1)..(7): CDRL2 of PD-1 mAb 8
KVSNRFS

SEQ ID NO: 168 - protein, 9 aa, Mus musculus
  MISC_FEATURE (1)..(9): CDRL3 of PD-1 mAb 8
SQSTHVPFT

SEQ ID NO: 169 - protein, 119 aa, Mus musculus
  MISC_FEATURE (1)..(119): VH Domain of PD-1 mAb 9
EVMLVESGGGLVKPGGSLKLSCAASGFTFSSYLVSWVRQTPEKRLEWVATISGGGGNTYYSDSVKGRFTISRDNAKNTLYLQISSLRSEDTALYYCARYGFDGAWFAYWGQGTLVTVSS

SEQ ID NO: 170 - DNA, 357 bp, Mus musculus
  misc_feature (1)..(357): Polynucleotide Encoding the VH Domain of PD-1 mAb 9
gaagtgatgctggtggagtctgggggaggcttagtgaagcctggagggtccctgaaactctcctgtgcagcctctggattcactttcagtagttatcttgtgtcttgggttcgccagactccggagaagaggctggagtgggtcgcaaccattagtggtggtggtggtaacacctactattcagacagtgtgaagggtcgattcaccatctccagagacaatgccaagaacaccctgtacctgcaaatcagcagtctgaggtctgaggacacggccttgtattactgtgcaaggtatggtttcgacggcgcctggtttgcttactggggccaagggactctggtcactgtctcttcc

SEQ ID NO: 171 - protein, 5 aa, Mus musculus
  MISC_FEATURE (1)..(5): CDRH1 of PD-1 mAb 9
SYLVS

SEQ ID NO: 172 - protein, 17 aa, Mus musculus
  MISC_FEATURE (1)..(17): CDRH2 of PD-1 mAb 9
TISGGGGNTYYSDSVKG

SEQ ID NO: 173 - protein, 10 aa, Mus musculus
  MISC_FEATURE (1)..(10): CDRH3 of PD-1 mAb 9
YGFDGAWFAY

SEQ ID NO: 174 - protein, 107 aa, Mus musculus
  MISC_FEATURE (1)..(107): VL Domain of PD-1 mAb 9
DIQMTQSPASLSASVGDIVTITCRASENIYSYLAWYQQKQEKSPQLLVYNAKTLAAGVPSRFSGSGSGTQFSLTINSLQPEDFGNYYCQHHYAVPWTFGGGTRLEIT

SEQ ID NO: 175 - DNA, 321 bp, Mus musculus
  misc_feature (1)..(321): Polynucleotide Encoding the VL Domain of PD-1 mAb 9
gacatccagatgactcagtctccagcctccctatctgcatctgtgggagatattgtcaccatcacatgtcgagcaagtgagaatatttacagttatttagcatggtatcagcagaaacaggaaaaatctcctcagctcctggtctataatgcaaaaaccttggcagcaggtgtgccatcaaggttcagtggcagtggatcaggcacacagttttctctgaccatcaacagcctgcagcctgaagattttgggaattattactgtcagcatcattatgctgttccgtggacgttcggtggaggcaccagactggaaatcaca

SEQ ID NO: 176 - protein, 11 aa, Mus musculus
  MISC_FEATURE (1)..(11): CDRL1 of PD-1 mAb 9
RASENIYSYLA

SEQ ID NO: 177 - protein, 7 aa, Mus musculus
  MISC_FEATURE (1)..(7): CDRL2 of PD-1 mAb 9
NAKTLAA

SEQ ID NO: 178 - protein, 9 aa, Mus musculus
  MISC_FEATURE (1)..(9): CDRL3 of PD-1 mAb 9
QHHYAVPWT

SEQ ID NO: 179 - protein, 119 aa, Artificial Sequence
  VH Domain of hPD-1 mAb 9 VH1
EVQLVESGGGLVRPGGSLKLSCAASGFTFSSYLVSWVRQAPGKGLEWVATISGGGGNTYYSDSVKGRFTISRDNAKNSLYLQMNSLRAEDTATYYCARYGFDGAWFAYWGQGTLVTVSS

SEQ ID NO: 180 - DNA, 357 bp, Artificial Sequence
  Polynucleotide Encoding hPD-1 mAb 9 VH1
gaggtgcagctggtggaaagtgggggcggcctggtgcgacccgggggaagtctgaaactgtcctgtgcagcatcaggatttactttttcatcttatctcgtgtcttgggtaagacaagcacccggaaaaggcttggaatgggtggccactatctccggtggaggtggcaacacctactatagcgacagtgtcaagggaagatttaccatcagtcgcgacaacgctaagaatagcctgtacctccagatgaactccctgcgcgccgaggacaccgccacctattactgtgcacgctatggatttgacggcgcatggtttgcctactggggacagggcacattggtaaccgttagctcc

SEQ ID NO: 181 - protein, 119 aa, Artificial Sequence
  VH Domain of hPD-1 mAb 9 VH2
EVQLVESGGGLARPGGSLKLSCAASGFTFSSYLVGWVRQAPGKGLEWTATISGGGGNTYYSDSVKGRFTISRDNAKNSLYLQMNSARAEDTATYYCARYGFDGAWFAYWGQGTLVTVSS

SEQ ID NO: 182 - DNA, 357 bp, Artificial Sequence
  Polynucleotide Encoding hPD-1 mAb 9 VH2
gaggtgcagctggtggaaagtgggggcggcctggcgcgacccgggggaagtctgaaactgtcctgtgcagcatcaggatttactttttcatcttatctcgtgggctgggtaagacaagcacccggaaaaggcttggaatggacggccactatctccggtggaggtggcaacacctactatagcgacagtgtcaagggaagatttaccatcagtcgcgacaacgctaagaatagcctgtacctccagatgaactccgcacgcgccgaggacaccgccacctattactgtgcacgctatggatttgacggcgcatggtttgcctactggggacagggcacattggtaaccgttagctcc

SEQ ID NO: 183 - protein, 5 aa, Artificial Sequence
  CDRH1 of the VH Domain of hPD-1 mAb 9 VH2 Having a Serine to Glycine Amino Acid Substitution
SYLVG

SEQ ID NO: 184 - protein, 107 aa, Artificial Sequence
  VL Domain of hPD-1 mAb 9 VL1
DIQMTQSPSSLSASVGDRVTITCRASENIYSYLAWYQQKPGKAPKLLIYNAKTLAAGVPSRFSGSGSGTDFTLTISSLQPEDFATYYCQHHYAVPWTFGQGTKLEIK

SEQ ID NO: 185 - DNA, 321 bp, Artificial Sequence
  Polynucleotide Encoding hPD-1 mAb 9 VL1
gacattcagatgactcagtctcccagcagtctgtccgcatccgtgggggatcgggtcaccatcacctgccgtgcctcagaaaacatctattcatacctcgcctggtatcaacagaaacctggtaaagccccaaaattgctcatttacaacgccaagaccctcgcagctggcgtgccaagtaggttctcaggcagcggctcagggacagatttcaccctcaccatatcctcactgcagcccgaggattttgccacttactactgccagcatcattacgcagtgccctggaccttcggacaaggcactaagctcgagatcaaa

SEQ ID NO: 186 - protein, 107 aa, Artificial Sequence
  VL Domain of hPD-1 mAb 9 VL2
DIQMTQSPSSLSASVGDRVTITCRASENIYNYLAWYQQKPGKAPKLLIYDAKTLAAGVPSRFSGSGSGTDFTLTISSLQPEDFATYYCQHHYAVPWTFGQGTKLEIK

SEQ ID NO: 187 - DNA, 321 bp, Artificial Sequence
  Polynucleotide Encoding hPD-1 mAb 9 VL2
gacattcagatgactcagtctcccagcagtctgtccgcatccgtgggggatcgggtcaccatcacctgccgtgcctcagaaaacatctataactacctcgcctggtatcaacagaaacctggtaaagccccaaaattgctcatttacgacgccaagaccctcgcagctggcgtgccaagtaggttctcaggcagcggctcagggacagatttcaccctcaccatatcctcactgcagcccgaggattttgccacttactactgccagcatcattacgcagtgccctggaccttcggacaaggcactaagctcgagatcaaa

SEQ ID NO: 188 - protein, 11 aa, Artificial Sequence
  CDRL1 of the VL Domain of hPD-1 mAb 9 VL2
RASENIYNYLA

SEQ ID NO: 189 - protein, 7 aa, Artificial Sequence
  CDRL2 of the VL Domain of hPD-1 mAb 9 VL2
DAKTLAA

SEQ ID NO: 190 - protein, 116 aa, Mus musculus
  MISC_FEATURE (1)..(116): VH Domain of PD-1 mAb 10
EVILVESGGGLVKPGGSLKLSCAASGFTFSNYLMSWVRQTPEKRLEWVASISGGGSNIYYPDSVKGRFTISRDNAKNTLYLQMNSLRSEDTALYYCARQELAFDYWGQGTTLTVSS

SEQ ID NO: 191 - DNA, 348 bp, Mus musculus
  misc_feature (1)..(348): Polynucleotide Encoding the VH Domain of PD-1 mAb 10
gaagtgatactggtggagtctgggggaggcttagtgaagcctggagggtccctgaaactctcctgtgcagcctctggattcactttcagtaactatctcatgtcttgggttcgccagactccggagaagaggctggagtgggtcgcaagtattagtggtggtggtagtaatatctactatccagacagtgtgaagggtcgattcaccatatccagggacaatgccaagaacaccctgtacctgcaaatgaacagtctgaggtctgaggacacggccttgtattactgtgcaagacaagaactggcttttgactactggggccaaggcaccactctcacagtctcctcc

SEQ ID NO: 192 - protein, 5 aa, Mus musculus
  MISC_FEATURE (1)..(5): CDRH1 of PD-1 mAb 10
NYLMS

SEQ ID NO: 193 - protein, 17 aa, Mus musculus
  MISC_FEATURE (1)..(17): CDRH2 of PD-1 mAb 10
SISGGGSNIYYPDSVKG

SEQ ID NO: 194 - protein, 7 aa, Mus musculus
  MISC_FEATURE (1)..(7): CDRH3 of PD-1 mAb 10
QELAFDY

SEQ ID NO: 195 - protein, 107 aa, Mus musculus
  MISC_FEATURE (1)..(107): VL Domain of PD-1 mAb 10
DIQMTQTTSSLSASLGDRVTISCRTSQDISNFLNWYQQKPDGTIKLLIYYTSRLHSGVPSRFSGSGSGTDYSLTISNLEQEDIATYFCQQGSTLPWTFGGGTKLEII

SEQ ID NO: 196 - DNA, 321 bp, Mus musculus
  misc_feature (1)..(321): Polynucleotide Encoding the VL Domain of PD-1 mAb 10
gatatccagatgacacagactacatcctccctgtctgcctctctgggagacagagtcaccatcagttgcaggacaagtcaggacattagcaattttttaaactggtatcagcagaaaccagatggaactattaaactcctgatctactacacatcaagattacactcaggagtcccatcaaggttcagtggcagtgggtctggaacagattattctctcaccattagcaacctggagcaagaagatattgccacttacttttgccaacagggtagtacgcttccgtggacgttcggtggaggcaccaagctggaaatcata

SEQ ID NO: 197 - protein, 11 aa, Mus musculus
  MISC_FEATURE (1)..(11): CDRL1 of PD-1 mAb 10
RTSQDISNFLN

SEQ ID NO: 198 - protein, 7 aa, Mus musculus
  MISC_FEATURE (1)..(7): CDRL2 of PD-1 mAb 10
YTSRLHS

SEQ ID NO: 199 - protein, 9 aa, Mus musculus
  MISC_FEATURE (19)..(): CDRL3 of PD-1 mAb 10
QQGSTLPWT

SEQ ID NO: 200 - protein, 117 aa, Mus musculus
  MISC_FEATURE (1)..(117): VH Domain of PD-1 mAb 11
EVQLQQSGTVLARPGASVKMSCKTSGYTFTGYWMHWVKQRPGQGLKWMGAIYPGNSDTHYNQKFKGKAKLTAVTSASTAYMELSSLTNEDSAIYYCTTGTYSYFDVWGTGTTVTVSS

SEQ ID NO: 201 - DNA, 351 bp, Mus musculus
  misc_feature (1)..(351): Polynucleotide Encoding the VH Domain of PD-1 mAb 11
gaggttcagctccagcagtctgggactgtgctggcaaggcctggggcttcagtgaagatgtcctgcaagacttctggctacacatttaccggctactggatgcactgggtaaaacagaggcctggacagggtctgaaatggatgggggctatttatcctggaaatagtgatactcactacaaccagaagttcaagggcaaggccaaactgactgcagtcacatccgccagcactgcctacatggagctcagcagcctgacaaatgaggactctgcgatctattactgtactactgggacctactcgtacttcgatgtctggggcacagggaccacggtcaccgtctcctca

SEQ ID NO: 202 - protein, 5 aa, Mus musculus
  MISC_FEATURE (1)..(5): CDRH1 of PD-1 mAb 11
GYWMH

SEQ ID NO: 203 - protein, 17 aa, Mus musculus
  MISC_FEATURE (1)..(17): CDRH2 of PD-1 mAb 11
AIYPGNSDTHYNQKFKG

SEQ ID NO: 204 - protein, 8 aa, Mus musculus
  MISC_FEATURE (1)..(8): CDRH3 of PD-1 mAb 11
GTYSYFDV

SEQ ID NO: 205 - protein, 106 aa, Mus musculus
  MISC_FEATURE (1)..(106): VL Domain of PD-1 mAb 11
DILLTQSPAILSVSPGERVSFSCRASQSIGTSIHWYQHRTNGSPRLLIKYASESISGIPSRFSGSGSGTDFTLSINSVESEDIADYYCQQSNSWLTFGAGTKLELK

SEQ ID NO: 206 - DNA, 318 bp, Mus musculus
  misc_feature (1)..(318): Polynucleotide Encoding the VL Domain of PD-1 mAb 11
gacatcttgctgactcagtctccagccatcctgtctgtgagtccaggagaaagagtcagtttctcctgcagggccagtcagagcattggcacaagcatacactggtatcagcacagaacaaatggttctccaaggcttctcataaagtatgcttctgagtctatctctgggatcccttccaggtttagtggcagtggatcagggactgattttactcttagcatcaacagtgtggagtctgaagatattgcagattattactgtcaacaaagtaatagctggctcacgttcggtgctgggaccaagctggagctgaaa

SEQ ID NO: 207 - protein, 11 aa, Mus musculus
  MISC_FEATURE (1)..(11): CDRL1 of PD-1 mAb 11
RASQSIGTSIH

SEQ ID NO: 208 - protein, 7 aa, Mus musculus
  MISC_FEATURE (1)..(7): CDRL2 of PD-1 mAb 11
YASESIS

SEQ ID NO: 209 - protein, 8 aa, Mus musculus
  MISC_FEATURE (1)..(8): CDRL3 of PD-1 mAb 11
QQSNSWLT

SEQ ID NO: 210 - protein, 125 aa, Mus musculus
  MISC_FEATURE (1)..(125): VH Domain of PD-1 mAb 12
QGHLQQSGAELVRPGASVTLSCKASGFTFTDYEMHWVKQTPVHGLEWIGTIDPETGGTAYNQKFKGKAILTVDKSSTTTYMELRSLTSEDSAVFYCSRERITTVVEGAYWYFDVWGTGTTVTVSS

SEQ ID NO: 211 - DNA, 375 bp, Mus musculus
  misc_feature (1)..(375): Polynucleotide Encoding the VH Domain of PD-1 mAb 12
cagggtcacctgcagcagtctggggctgagctggtgaggcctggggcttcagtgacgctgtcctgcaaggcttcgggcttcacatttactgactatgagatgcactgggtgaaacagacacctgtgcatggcctggaatggattgggactattgatcctgaaactggtggtactgcctacaatcagaagttcaagggcaaggccatactgacagtagacaaatcttccactacaacctacatggagctccgcagcctgacatctgaggactctgccgtcttttattgttcaagagagaggattactacggttgttgagggggcatactggtacttcgatgtctggggcacagggaccacggtcaccgtctcctca

SEQ ID NO: 212 - protein, 5 aa, Mus musculus
  MISC_FEATURE (1)..(5): CDRH1 of PD-1 mAb 12
DYEMH

SEQ ID NO: 213 - protein, 17 aa, Mus musculus
  MISC_FEATURE (1)..(17): CDRH2 of PD-1 mAb 12
TIDPETGGTAYNQKFKG

SEQ ID NO: 214 - protein, 16 aa, Mus musculus
  MISC_FEATURE (1)..(16): CDRH3 of PD-1 mAb 12
ERITTVVEGAYWYFDV

SEQ ID NO: 215 - protein, 112 aa, Mus musculus
  MISC_FEATURE (1)..(112): VL Domain of PD-1 mAb 4
DVLMTQTPLSLPVSLGDQASISCRSSQNIVHSNGNTYLEWYLQKPGQSPKLLICKVSTRFSGVPDRFSGSGSGTDFTLKISRVEAEDLGVYYCFQGSHVPYTFGGGTKLEIK

SEQ ID NO: 216 - DNA, 336 bp, Mus musculus
  misc_feature (1)..(336): Polynucleotide Encoding the VL Domain of PD-1 mAb 12
gatgttttgatgacccagactccactctccctgcctgtcagtcttggagatcaagcctccatctcttgcagatctagtcagaacattgtacatagtaatggaaacacctatttagaatggtacctgcagaaaccaggccagtctccaaagctcctgatctgcaaagtttccacccgattttctggggtcccagacaggttcagtggcagtggatcagggacagatttcacactcaagatcagcagagtggaggctgaggatctgggagtttattattgctttcaaggttcacatgttccgtacacgttcggaggggggaccaagctggaaataaaa

SEQ ID NO: 217 - protein, 16 aa, Mus musculus
  MISC_FEATURE (1)..(16): CDRL1 of PD-1 mAb 12
RSSQNIVHSNGNTYLE

SEQ ID NO: 218 - protein, 7 aa, Mus musculus
  MISC_FEATURE (1)..(7): CDRL2 of PD-1 mAb 12
KVSTRFS

SEQ ID NO: 219 - protein, 9 aa, Mus musculus
  MISC_FEATURE (1)..(9): CDRL3 of PD-1 mAb 12
FQGSHVPYT

SEQ ID NO: 220 - protein, 121 aa, Mus musculus
  MISC_FEATURE (1)..(121): VH Domain of PD-1 mAb 13
EVMLVESGGGLVKPGGSLKLSCAASGFTFSSHTMSWVRQTPEKRLEWVATISGGGSNIYYPDSVKGRFTISRDNAKNTLYLQMSSLRSEDTALYYCARQAYYGNYWYFDVWGTGTTVTVSS

SEQ ID NO: 221 - DNA, 363 bp, Mus musculus
  misc_feature (1)..(363): Polynucleotide Encoding the VH Domain of PD-1 mAb 13
gaagtgatgctggtggagtctgggggaggcttagtgaagcctggagggtccctgaaactctcctgtgcagcctctggattcactttcagtagccataccatgtcttgggttcgccagactccggagaagaggctggagtgggtcgcaaccattagtggtggtggttctaatatctactatccagacagtgtgaagggtcgattcaccatctccagagacaatgccaagaacaccctgtacctgcaaatgagcagtctgaggtctgaggacacggccttgtattactgtgcaagacaagcttactacggtaattactggtacttcgatgtctggggcacagggaccacggtcaccgtctcctcc

SEQ ID NO: 222 - protein, 5 aa, Mus musculus
  MISC_FEATURE (1)..(5): CDRH1 of PD-1 mAb 13
SHTMS

SEQ ID NO: 223 - protein, 17 aa, Mus musculus
  MISC_FEATURE (1)..(17): CDRH2 of PD-1 mAb 13
TISGGGSNIYYPDSVKG

SEQ ID NO: 224 - protein, 12 aa, Mus musculus
  MISC_FEATURE (1)..(12): CDRH3 of PD-1 mAb 13
QAYYGNYWYFDV

SEQ ID NO: 225 - protein, 107 aa, Mus musculus
  MISC_FEATURE (1)..(107): VL Domain of PD-1 mAb 13
DIQMTQSPATQSASLGESVTITCLASQTIGTWLAWYQQKPGKSPQLLIYAATSLADGVPSRFSGSGSGTKFSFKISSLQAEDFVSYYCQQLDSIPWTFGGGTKLEIK

SEQ ID NO: 226 - DNA, 321 bp, Mus musculus
  misc_feature (1)..(321): Polynucleotide Encoding the VL Domain of PD-1 mAb 13
gacattcagatgacccagtctcctgccacccagtctgcatctctgggagaaagtgtcaccatcacgtgcctggcaagtcagaccattggtacatggttagcatggtatcagcagaaaccagggaaatctcctcagctcctgatttatgctgcaaccagcttggcagatggggtcccatcaaggttcagtggtagtggatctggcacaaaattttctttcaagatcagcagcctacaggctgaagattttgtaagttattactgtcaacaacttgacagtattccgtggacgttcggtggaggcaccaagctggaaatcaaa

SEQ ID NO: 227 - protein, 11 aa, Mus musculus
  MISC_FEATURE (1)..(11): CDRL1 of PD-1 mAb 13
LASQTIGTWLA

SEQ ID NO: 228 - protein, 7 aa, Mus musculus
  MISC_FEATURE (1)..(7): CDRL2 of PD-1 mAb 13
AATSLAD

SEQ ID NO: 229 - protein, 9 aa, Mus musculus
  MISC_FEATURE (1)..(9): CDRL3 of PD-1 mAb 13
QQLDSIPWT

SEQ ID NO: 230 - protein, 117 aa, Mus musculus
  MISC_FEATURE (1)..(117): VH Domain of PD-1 mAb 14
QVQLQQPGAELVKPGASVKMSCKASGYNFISYWITWVKQRPGQGLQWIGNIYPGTDGTTYNEKFKSKATLTVDTSSSTAYMHLSRLTSEDSAVYYCATGLHWYFDVWGTGTTVTVSS

SEQ ID NO: 231 - DNA, 351 bp, Mus musculus
  misc_feature (1)..(351): Polynucleotide Encoding the VH Domain of PD-1 mAb 14
caggtccaactgcagcagcctggggctgagcttgtgaagcctggggcttcagtgaagatgtcctgcaaggcttctggctacaacttcatcagctactggataacctgggtgaaacagaggcctggacaaggccttcagtggattggaaatatttatcctggtactgatggtactacctacaatgagaagttcaagagcaaggccacactgactgtagacacatcctccagcacagcctacatgcacctcagtcgcctgacatctgaggactctgcggtctattactgtgcaactgggctacactggtacttcgatgtctggggcacagggaccacggtcaccgtctcctcc

SEQ ID NO: 232 - protein, 5 aa, Mus musculus
  MISC_FEATURE (1)..(5): CDRH1 of PD-1 mAb 14
SYWIT

SEQ ID NO: 233 - protein, 17 aa, Mus musculus
  MISC_FEATURE (1)..(17): CDRH2 of PD-1 mAb 14
NIYPGTDGTTYNEKFKS

SEQ ID NO: 234 - protein, 8 aa, Mus musculus
  MISC_FEATURE (1)..(8): CDRH3 of PD-1 mAb 14
GLHWYFDV

SEQ ID NO: 235 - protein, 107 aa, Mus musculus
  MISC_FEATURE (1)..(107): VL Domain of PD-1 mAb 14
DIVMTQSQKFMSTSVGDRVSVTCKASQSVGTNVAWYQQKPGQSPKALIYSASSRFSGVPDRFTGSGSGTDFTLTISNVQSEDLAEYFCQQYNSYPYTFGGGTKLEIK

SEQ ID NO: 236 - DNA, 321 bp, Mus musculus
  misc_feature (1)..(321): Polynucleotide Encoding the VL Domain of PD-1 mAb 14
gacattgtgatgacccagtctcaaaaattcatgtccacatcagtaggagacagggtcagtgtcacctgcaaggccagtcagagtgtgggtactaatgtagcctggtatcaacagaagcccggtcaatctcctaaagcactgatttactcggcatcctcccgattcagtggcgtccctgatcgcttcacaggcagtggatctgggacagatttcactctcaccatcagtaatgtgcagtctgaagacttggcagagtatttctgtcagcaatataacagctatccgtacacgttcggaggggggaccaagctggaaataaaa

SEQ ID NO: 237 - protein, 11 aa, Mus musculus
  MISC_FEATURE (1)..(11): CDRL1 of PD-1 mAb 14
KASQSVGTNVA

SEQ ID NO: 238 - protein, 7 aa, Mus musculus
  MISC_FEATURE (1)..(7): CDRL2 of PD-1 mAb 14
SASSRFS

SEQ ID NO: 239 - protein, 9 aa, Mus musculus
  MISC_FEATURE (1)..(9): CDRL3 of PD-1 mAb 14
QQYNSYPYT

SEQ ID NO: 240 - protein, 117 aa, Mus musculus
  MISC_FEATURE (1)..(117): VH Domain of PD-1 mAb 15
EVMLVESGGGLVKPGGSLKLSCAASGFIFSSYLISWVRQTPEKRLEWVAAISGGGADTYYADSVKGRFTISRDNAKNTLYLQMSSLRSEDTALYYCTRRGTYAMDYWGQGTSVTVSS

SEQ ID NO: 241 - DNA, 351 bp, Mus musculus
  misc_feature (1)..(351): Polynucleotide Encoding the VH Domain of PD-1 mAb 15
gaagtgatgctggtggagtctgggggaggcttagtgaagcctggagggtccctgaaactctcctgtgcagcctctggattcattttcagtagctatctcatctcttgggttcgccagactccggagaagaggctggagtgggtcgctgccattagtggtggtggtgctgacacctactatgccgacagtgtgaagggtcgattcaccatctccagagacaatgccaagaacaccctgtatctgcaaatgagcagtctgaggtctgaggacacggccttatattactgtacaagacgagggacctatgctatggactactggggtcaaggaacctcagtcaccgtctcctcc

SEQ ID NO: 242 - protein, 5 aa, Mus musculus
  MISC_FEATURE (1)..(5): CDRH1 of PD-1 mAb 15
SYLIS

SEQ ID NO: 243 - protein, 17 aa, Mus musculus
  MISC_FEATURE (1)..(17): CDRH2 of PD-1 mAb 15
AISGGGADTYYADSVKG

SEQ ID NO: 244 - protein, 8 aa, Mus musculus
  MISC_FEATURE (1)..(8): CDRH3 of PD-1 mAb 15
RGTYAMDY

SEQ ID NO: 245 - protein, 107 aa, Mus musculus
  MISC_FEATURE (1)..(107): VL Domain of PD-1 mAb 15
DIQMTQSPASQSASLGESVTITCLASQTIGTWLAWYQQKPGKSPQLLIYAATSLADGVPSRFSGSGSGTKFSFKISSLQAEDFVNYYCQQLYSIPWTFGGGTKLEIK

SEQ ID NO: 246 - DNA, 321 bp, Mus musculus
  misc_feature (1)..(321): Polynucleotide Encoding the VL Domain of PD-1 mAb 15
gacattcagatgacccagtctcccgcctcccagtctgcatctctgggagaaagtgtcaccatcacatgcctggcaagtcagaccattggtacatggttagcatggtatcagcagaaaccagggaaatctcctcagctcctgatttatgctgcaaccagcttggcagatggggtcccatcaaggttcagtggtagtggatctggcacaaaattttctttcaagatcagcagcctacaggctgaagattttgtaaattattactgtcaacaactttacagtattccgtggacgttcggtggaggcaccaagctggaaatcaaa

SEQ ID NO: 247 - protein, 11 aa, Mus musculus
  MISC_FEATURE (1)..(11): CDRL1 of PD-1 mAb 15
LASQTIGTWLA

SEQ ID NO: 248 - protein, 7 aa, Mus musculus
  MISC_FEATURE (1)..(7): CDRL2 of PD-1 mAb 15
AATSLAD

SEQ ID NO: 249 - protein, 9 aa, Mus musculus
  MISC_FEATURE (1)..(9): CDRL3 of PD-1 mAb 15
QQLYSIPWT

SEQ ID NO: 250 - protein, 117 aa, Artificial Sequence
  VH Domain of hPD-1 mAb 15 VH1
EVQLVESGGGLVRPGGSLRLSCAASGFTFSSYLISWVRQAPGKGLEWVAAISGGGADTYYADSVKGRFTISRDNAKNSLYLQMNSLRAEDTATYYCARRGTYAMDYWGQGTLVTVSS

SEQ ID NO: 251 - DNA, 351 bp, Artificial Sequence
  Polynucleotide Encoding hPD-1 mAb 15 VH1
gaagtgcaactggttgaaagtggcggcgggctggtgcggccaggtggttcactcagactgtcttgtgcagcttcaggctttacattctcctcttatcttatctcttgggtgcgccaagccccaggtaagggccttgaatgggtcgccgccattagtgggggtggtgccgatacatattatgccgacagcgtcaagggacgtttcaccatcagcagggacaacgccaagaatagcctttacctgcagatgaactcacttagagctgaagacaccgctacttattactgtgcccggcgcgggacttacgctatggactattggggccagggcaccttggtcactgtctcatcc

SEQ ID NO: 252 - protein, 107 aa, Artificial Sequence
  VH Domain of hPD-1 mAb 15 VL1
DIQMTQSPSSLSASVGDRVTITCLASQTIGTWLAWYQQKPGKAPKLLIYAATSLADGVPSRFSGSGSGTDFTFTISSLQPEDFATYYCQQLYSIPWTFGQGTKLEIK

SEQ ID NO: 253 - DNA, 321 bp, Artificial Sequence
  Polynucleotide encoding hPD-1 mAb 15 VL1
gatatccagatgacccagtctcccagctctctcagtgcaagcgtaggcgaccgtgtgaccatcacctgtctggccagtcagaccattggaacctggctcgcctggtatcagcagaaacctggcaaggcccctaagctgctgatttacgccgccacctccctcgcagatggagtgccctcccgatttagcgggtccgggtccggcaccgacttcacattcacaatcagcagcctccagcccgaggatttcgctacatactactgtcaacagctctactccattccatggacctttggtcagggtactaaactggagatcaaa

SEQ ID NO: 254 - protein, 98 aa, Homo sapiens
  MISC_FEATURE (1)..(98): Human IgG4 CH1 Domain
ASTKGPSVFPLAPCSRSTSESTAALGCLVKDYFPEPVTVSWNSGALTSGVHTFPAVLQSSGLYSLSSVVTVPSSSLGTKTYTCNVDHKPSNTKVDKRV

SEQ ID NO: 255 - protein, 329 aa, Artificial Sequence
  IgG1 Humanized Antibody Heavy Chain
ASTKGPSVFPLAPSSKSTSGGTAALGCLVKDYFPEPVTVSWNSGALTSGVHTFPAVLQSSGLYSLSSVVTVPSSSLGTQTYICNVNHKPSNTKVDKRVEPKSCDKTHTCPPCPAPEAAGGPSVFLFPPKPKDTLMISRTPEVTCVVVDVSHEDPEVKFNWYVDGVEVHNAKTKPREEQYNSTYRVVSVLTVLHQDWLNGKEYKCKVSNKALPAPIEKTISKAKGQPREPQVYTLPPSREEMTKNQVSLTCLVKGFYPSDIAVEWESNGQPENNYKTTPPVLDSDGSFFLYSKLTVDKSRWQQGNVFSCSVMHEALHNHYTQKSLSLSPG

SEQ ID NO: 256 - protein, 326 aa, Artificial Sequence
  IgG4 Humanized Antibody Heavy Chain with Stabilized Hinge Region
ASTKGPSVFPLAPCSRSTSESTAALGCLVKDYFPEPVTVSWNSGALTSGVHTFPAVLQSSGLYSLSSVVTVPSSSLGTKTYTCNVDHKPSNTKVDKRVESKYGPPCPPCPAPEFLGGPSVFLFPPKPKDTLMISRTPEVTCVVVDVSQEDPEVQFNWYVDGVEVHNAKTKPREEQFNSTYRVVSVLTVLHQDWLNGKEYKCKVSNKGLPSSIEKTISKAKGQPREPQVYTLPPSQEEMTKNQVSLTCLVKGFYPSDIAVEWESNGQPENNYKTTPPVLDSDGSFFLYSRLTVDKSRWQEGNVFSCSVMHEALHNHYTQKSLSLSLG

SEQ ID NO: 257 - protein, 98 aa, Homo sapiens
  MISC_FEATURE (1)..(98): Human IgG2 CH1 Domain
ASTKGPSVFPLAPCSRSTSESTAALGCLVKDYFPEPVTVSWNSGALTSGVHTFPAVLQSSGLYSLSSVVTVPSSNFGTQTYTCNVDHKPSNTKVDKTV

SEQ ID NO: 258 - protein, 217 aa, Artificial Sequence
  IgG1 Sequence for the CH2 and CH3 Domains
  MISC_FEATURE (217)..(217): Xaa is a lysine (K) or is absent
APEAAGGPSVFLFPPKPKDTLYITREPEVTCVVVDVSHEDPEVKFNWYVDGVEVHNAKTKPREEQYNSTYRVVSVLTVLHQDWLNGKEYKCKVSNKALPAPIEKTISKAKGQPREPQVYTLPPSREEMTKNQVSLTCLVKGFYPSDIAVEWESNGQPENNYKTTPPVLDSDGSFFLYSKLTVDKSRWQQGNVFSCSVMHEALHNHYTQKSLSLSPGX

SEQ ID NO: 259 - protein, 217 aa, Artificial Sequence
  IgG4 Sequence for the CH2 and CH3 Domains
  MISC_FEATURE (217)..(217): Xaa is a lysine (K) or is absent
APEFLGGPSVFLFPPKPKDTLYITREPEVTCVVVDVSQEDPEVQFNWYVDGVEVHNAKTKPREEQFNSTYRVVSVLTVLHQDWLNGKEYKCKVSNKGLPSSIEKTISKAKGQPREPQVYTLPPSQEEMTKNQVSLTCLVKGFYPSDIAVEWESNGQPENNYKTTPPVLDSDGSFFLYSRLTVDKSRWQEGNVFSCSVMHEALHNHYTQKSLSLSLGX

SEQ ID NO: 260 - protein, 217 aa, Artificial Sequence
  Wild-type and Variant Human IgG1 CH2 and CH3 Domains
  MISC_FEATURE (4)..(5): Xaa4 and Xaa5 are both L (wild type), or are both A (decreased FcgammaR binding)
  MISC_FEATURE (22)..(26): Xaa22, Xaa24 and Xaa26 respectively are M, S and T (wild type), or are Y, T and E (extended half-life)
  MISC_FEATURE (136)..(177): Xaa136, Xaa138, and Xaa177 respectively are: T, L and Y (wild type), or are W, L and Y (knob), or S, A and V (hole)
  MISC_FEATURE (204)..(205): Xaa204 and Xaa205 respectively are N and H (wild type), or are N and R (no protein A binding), or A and K (no protein A binding)
  MISC_FEATURE (217)..(217): Xaa217 is K or is absent
APEXXGGPSVFLFPPKPKDTLXIXRXPEVTCVVVDVSHEDPEVKFNWYVDGVEVHNAKTKPREEQYNSTYRVVSVLTVLHQDWLNGKEYKCKVSNKALPAPIEKTISKAKGQPREPQVYTLPPSREEMTKNQVSLXCXVKGFYPSDIAVEWESNGQPENNYKTTPPVLDSDGSFFLXSKLTVDKSRWQQGNVFSCSVMHEALHXXYTQKSLSLSPGX

SEQ ID NO: 261 - protein, 6 aa, Artificial Sequence
  Alternative Linker 2
LGGGSG

SEQ ID NO: 262 - protein, 11 aa, Artificial Sequence
  Linker 3
GGGSGGGSGGG

SEQ ID NO: 263 - protein, 13 aa, Artificial Sequence
  Linker 3
GGGDKTHTCPPCP

SEQ ID NO: 264 - protein, 218 aa, Artificial Sequence
  Light Chain of a Humanized PD-1 Antibody (hPD-1 mAb 7(1.2))
EIVLTQSPATLSLSPGERATLSCRASESVDNYGMSFMNWFQQKPGQPPKLLIHAASNQGSGVPSRFSGSGSGTDFTLTISSLEPEDFAVYFCQQSKEVPYTFGGGTKVEIKRTVAAPSVFIFPPSDEQLKSGTASVVCLLNNFYPREAKVQWKVDNALQSGNSQESVTEQDSKDSTYSLSSTLTLSKADYEKHKVYACEVTHQGLSSPVTKSFNRGEC

SEQ ID NO: 265 - protein, 448 aa, Artificial Sequence
  Heavy Chain of a Humanized Antibody ((hPD-1 mAb 7(1.2))
QVQLVQSGAEVKKPGASVKVSCKASGYSFTSYWMNWVRQAPGQGLEWIGVIHPSDSETWLDQKFKDRVTITVDKSTSTAYMELSSLRSEDTAVYYCAREHYGTSPFAYWGQGTLVTVSSASTKGPSVFPLAPSSKSTSGGTAALGCLVKDYFPEPVTVSWNSGALTSGVHTFPAVLQSSGLYSLSSVVTVPSSSLGTQTYICNVNHKPSNTKVDKRVEPKSCDKTHTCPPCPAPEAAGGPSVFLFPPKPKDTLMISRTPEVTCVVVDVSHEDPEVKFNWYVDGVEVHNAKTKPREEQYNSTYRVVSVLTVLHQDWLNGKEYKCKVSNKALPAPIEKTISKAKGQPREPQVYTLPPSREEMTKNQVSLTCLVKGFYPSDIAVEWESNGQPENNYKTTPPVLDSDGSFFLYSKLTVDKSRWQQGNVFSCSVMHEALHNHYTQKSLSLSPG

SEQ ID NO: 266 - protein, 445 aa, Artificial Sequence
  Heavy Chain of a Humanized Antibody ((hPD-1 mAb 7(1.2))
QVQLVQSGAEVKKPGASVKVSCKASGYSFTSYWMNWVRQAPGQGLEWIGVIHPSDSETWLDQKFKDRVTITVDKSTSTAYMELSSLRSEDTAVYYCAREHYGTSPFAYWGQGTLVTVSSASTKGPSVFPLAPCSRSTSESTAALGCLVKDYFPEPVTVSWNSGALTSGVHTFPAVLQSSGLYSLSSVVTVPSSSLGTKTYTCNVDHKPSNTKVDKRVESKYGPPCPPCPAPEFLGGPSVFLFPPKPKDTLMISRTPEVTCVVVDVSQEDPEVQFNWYVDGVEVHNAKTKPREEQFNSTYRVVSVLTVLHQDWLNGKEYKCKVSNKGLPSSIEKTISKAKGQPREPQVYTLPPSQEEMTKNQVSLTCLVKGFYPSDIAVEWESNGQPENNYKTTPPVLDSDGSFFLYSRLTVDKSRWQEGNVFSCSVMHEALHNHYTQKSLSLSLG

SEQ ID NO: 267 - protein, 501 aa, Artificial Sequence
  First and Third Polypeptide Chains of DART A
  MISC_FEATURE (34)..(34): Xaa34 is A or G
  MISC_FEATURE (307)..(307): Xaa307 is Y or M
  MISC_FEATURE (309)..(309): Xaa309 is T or S
  MISC_FEATURE (311)..(311): Xaa311 is E or T
DIVMTQTPLSLSVTPGQPASISCKSSQSLLHSDXKTYLNWLLQKPGQPPERLIYLVSELDSGVPDRFSGSGSGTDFTLKISRVEAEDVGVYYCWQGTHFPYTFGGGTKVEIKGGGSGGGGQVQLVQSGAEVKKPGASVKVSCKASGYSFTSYWMNWVRQAPGQGLEWIGVIHPSDSETWLDQKFKDRVTITVDKSTSTAYMELSSLRSEDTAVYYCAREHYGTSPFAYWGQGTLVTVSSGGCGGGEVAACEKEVAALEKEVAALEKEVAALEKESKYGPPCPPCPAPEFLGGPSVFLFPPKPKDTLXIXRXPEVTCVVVDVSQEDPEVQFNWYVDGVEVHNAKTKPREEQFNSTYRVVSVLTVLHQDWLNGKEYKCKVSNKGLPSSIEKTISKAKGQPREPQVYTLPPSQEEMTKNQVSLTCLVKGFYPSDIAVEWESNGQPENNYKTTPPVLDSDGSFFLYSRLTVDKSRWQEGNVFSCSVMHEALHNHYTQKSLSLSLG

SEQ ID NO: 268 - protein, 273 aa, Artificial Sequence
  Second and Fourth Polypeptide Chains of DART A
EIVLTQSPATLSLSPGERATLSCRASESVDNYGMSFMNWFQQKPGQPPKLLIHAASNQGSGVPSRFSGSGSGTDFTLTISSLEPEDFAVYFCQQSKEVPYTFGGGTKVEIKGGGSGGGGQVQLVQSGAEVKKPGASVKVSCKASGYTFTNYGMNWVRQAPGQGLEWMGWINTYTGESTYADDFEGRFVFSMDTSASTAYLQISSLKAEDTAVYYCARESLYDYYSMDYWGQGTTVTVSSGGCGGGKVAACKEKVAALKEKVAALKEKVAALKE

SEQ ID NO: 269 - protein, 571 aa, Artificial Sequence
  First and Third Polypeptide Chains of DART D
EIVLTQSPATLSLSPGERATLSCRASESVDNYGMSFMNWFQQKPGQPPKLLIHAASNQGSGVPSRFSGSGSGTDFTLTISSLEPEDFAVYFCQQSKEVPYTFGGGTKVEIKGGGSGGGGQVQLVQSGAEVKKPGASVKVSCKASGYTFTNYGMNWVRQAPGQGLEWMGWINTYTGESTYADDFEGRFVFSMDTSASTAYLQISSLKAEDTAVYYCARESLYDYYSMDYWGQGTTVTVSSLGGGSGASTKGPSVFPLAPCSRSTSESTAALGCLVKDYFPEPVTVSWNSGALTSGVHTFPAVLQSSGLYSLSSVVTVPSSSLGTKTYTCNVDHKPSNTKVDKRVESKYGPPCPPCPAPEFLGGPSVFLFPPKPKDTLYITREPEVTCVVVDVSQEDPEVQFNWYVDGVEVHNAKTKPREEQFNSTYRVVSVLTVLHQDWLNGKEYKCKVSNKGLPSSIEKTISKAKGQPREPQVYTLPPSQEEMTKNQVSLTCLVKGFYPSDIAVEWESNGQPENNYKTTPPVLDSDGSFFLYSRLTVDKSRWQEGNVFSCSVMHEALHNHYTQKSLSLSLG

SEQ ID NO: 270 - protein, 352 aa, Artificial Sequence
  Second and Fourth Polypeptide Chains of DART D
DIVMTQTPLSLSVTPGQPASISCKSSQSLLHSDAKTYLNWLLQKPGQPPERLIYLVSELDSGVPDRFSGSGSGTDFTLKISRVEAEDVGVYYCWQGTHFPYTFGGGTKVEIKGGGSGGGGQVQLVQSGAEVKKPGASVKVSCKASGYSFTSYWMNWVRQAPGQGLEWIGVIHPSDSETWLDQKFKDRVTITVDKSTSTAYMELSSLRSEDTAVYYCAREHYGTSPFAYWGQGTLVTVSSLGGGSGRTVAAPSVFIFPPSDEQLKSGTASVVCLLNNFYPREAKVQWKVDNALQSGNSQESVTEQDSKDSTYSLSSTLTLSKADYEKHKVYACEVTHQGLSSPVTKSFNRGEC

SEQ ID NO: 271 - protein, 571 aa, Artificial Sequence
  First and Third Polypeptide Chains of DART E
DIVMTQTPLSLSVTPGQPASISCKSSQSLLHSDAKTYLNWLLQKPGQPPERLIYLVSELDSGVPDRFSGSGSGTDFTLKISRVEAEDVGVYYCWQGTHFPYTFGGGTKVEIKGGGSGGGGQVQLVQSGAEVKKPGASVKVSCKASGYSFTSYWMNWVRQAPGQGLEWIGVIHPSDSETWLDQKFKDRVTITVDKSTSTAYMELSSLRSEDTAVYYCAREHYGTSPFAYWGQGTLVTVSSLGGGSGASTKGPSVFPLAPCSRSTSESTAALGCLVKDYFPEPVTVSWNSGALTSGVHTFPAVLQSSGLYSLSSVVTVPSSSLGTKTYTCNVDHKPSNTKVDKRVESKYGPPCPPCPAPEFLGGPSVFLFPPKPKDTLYITREPEVTCVVVDVSQEDPEVQFNWYVDGVEVHNAKTKPREEQFNSTYRVVSVLTVLHQDWLNGKEYKCKVSNKGLPSSIEKTISKAKGQPREPQVYTLPPSQEEMTKNQVSLTCLVKGFYPSDIAVEWESNGQPENNYKTTPPVLDSDGSFFLYSRLTVDKSRWQEGNVFSCSVMHEALHNHYTQKSLSLSLG

SEQ ID NO: 272 - protein, 352 aa, Artificial Sequence
  Second and Fourth Polypeptide Chains of DART E
EIVLTQSPATLSLSPGERATLSCRASESVDNYGMSFMNWFQQKPGQPPKLLIHAASNQGSGVPSRFSGSGSGTDFTLTISSLEPEDFAVYFCQQSKEVPYTFGGGTKVEIKGGGSGGGGQVQLVQSGAEVKKPGASVKVSCKASGYTFTNYGMNWVRQAPGQGLEWMGWINTYTGESTYADDFEGRFVFSMDTSASTAYLQISSLKAEDTAVYYCARESLYDYYSMDYWGQGTTVTVSSLGGGSGRTVAAPSVFIFPPSDEQLKSGTASVVCLLNNFYPREAKVQWKVDNALQSGNSQESVTEQDSKDSTYSLSSTLTLSKADYEKHKVYACEVTHQGLSSPVTKSFNRGEC

SEQ ID NO: 273 - protein, 448 aa, Artificial Sequence
  First Polypeptide Chain of DART F
QVQLVQSGAEVKKPGASVKVSCKASGYSFTSYWMNWVRQAPGQGLEWIGVIHPSDSETWLDQKFKDRVTITVDKSTSTAYMELSSLRSEDTAVYYCAREHYGTSPFAYWGQGTLVTVSSASTKGPSVFPLAPSSKSTSGGTAALGCLVKDYFPEPVTVSWNSGALTSGVHTFPAVLQSSGLYSLSSVVTVPSSSLGTQTYICNVNHKPSNTKVDKRVEPKSCDKTHTCPPCPAPEAAGGPSVFLFPPKPKDTLYITREPEVTCVVVDVSHEDPEVKFNWYVDGVEVHNAKTKPREEQYNSTYRVVSVLTVLHQDWLNGKEYKCKVSNKALPAPIEKTISKAKGQPREPQVYTLPPSREEMTKNQVSLSCAVKGFYPSDIAVEWESNGQPENNYKTTPPVLDSDGSFFLVSKLTVDKSRWQQGNVFSCSVMHEALHAKYTQKSLSLSPG

SEQ ID NO: 274 - protein, 218 aa, Artificial Sequence; identical to SEQ ID NO: 264
  Second and Fifth Polypeptide Chains of DART F

SEQ ID NO: 275 - protein, 732 aa, Artificial Sequence
  Third Polypeptide Chain of DART F
QVQLVQSGAEVKKPGASVKVSCKASGYSFTSYWMNWVRQAPGQGLEWIGVIHPSDSETWLDQKFKDRVTITVDKSTSTAYMELSSLRSEDTAVYYCAREHYGTSPFAYWGQGTLVTVSSASTKGPSVFPLAPSSKSTSGGTAALGCLVKDYFPEPVTVSWNSGALTSGVHTFPAVLQSSGLYSLSSVVTVPSSSLGTQTYICNVNHKPSNTKVDKRVEPKSCDKTHTCPPCPAPEAAGGPSVFLFPPKPKDTLYITREPEVTCVVVDVSHEDPEVKFNWYVDGVEVHNAKTKPREEQYNSTYRVVSVLTVLHQDWLNGKEYKCKVSNKALPAPIEKTISKAKGQPREPQVYTLPPSREEMTKNQVSLWCLVKGFYPSDIAVEWESNGQPENNYKTTPPVLDSDGSFFLYSKLTVDKSRWQQGNVFSCSVMHEALHNHYTQKSLSLSPGGGGSGGGSGGGDIVMTQTPLSLSVTPGQPASISCKSSQSLLHSDAKTYLNWLLQKPGQPPERLIYLVSELDSGVPDRFSGSGSGTDFTLKISRVEAEDVGVYYCWQGTHFPYTFGGGTKVEIKGGGSGGGGQVQLVQSGAEVKKPGASVKVSCKASGYSFTSYWMNWVRQAPGQGLEWIGVIHPSDSETWLDQKFKDRVTITVDKSTSTAYMELSSLRSEDTAVYYCAREHYGTSPFAYWGQGTLVTVSSGGCGGGEVAALEKEVAALEKEVAALEKEVAALEK

SEQ ID NO: 276 - protein, 273 aa, Artificial Sequence
  Fourth Polypeptide Chain of DART F
EIVLTQSPATLSLSPGERATLSCRASESVDNYGMSFMNWFQQKPGQPPKLLIHAASNQGSGVPSRFSGSGSGTDFTLTISSLEPEDFAVYFCQQSKEVPYTFGGGTKVEIKGGGSGGGGQVQLVQSGAEVKKPGASVKVSCKASGYTFTNYGMNWVRQAPGQGLEWMGWINTYTGESTYADDFEGRFVFSMDTSASTAYLQISSLKAEDTAVYYCARESLYDYYSMDYWGQGTTVTVSSGGCGGGKVAALKEKVAALKEKVAALKEKVAALKE

SEQ ID NO: 277 - protein, 449 aa, Artificial Sequence
  First Polypeptide Chain of DART G
QVQLVQSGAEVKKPGASVKVSCKASGYTFTNYGMNWVRQAPGQGLEWMGWINTYTGESTYADDFEGRFVFSMDTSASTAYLQISSLKAEDTAVYYCARESLYDYYSMDYWGQGTTVTVSSASTKGPSVFPLAPSSKSTSGGTAALGCLVKDYFPEPVTVSWNSGALTSGVHTFPAVLQSSGLYSLSSVVTVPSSSLGTQTYICNVNHKPSNTKVDKRVEPKSCDKTHTCPPCPAPEAAGGPSVFLFPPKPKDTLYITREPEVTCVVVDVSHEDPEVKFNWYVDGVEVHNAKTKPREEQYNSTYRVVSVLTVLHQDWLNGKEYKCKVSNKALPAPIEKTISKAKGQPREPQVYTLPPSREEMTKNQVSLSCAVKGFYPSDIAVEWESNGQPENNYKTTPPVLDSDGSFFLVSKLTVDKSRWQQGNVFSCSVMHEALHAKYTQKSLSLSPG

SEQ ID NO: 278 - protein, 219 aa, Artificial Sequence
  Second and Fifth Polypeptide Chain of DART G
DIVMTQTPLSLSVTPGQPASISCKSSQSLLHSDAKTYLNWLLQKPGQPPERLIYLVSELDSGVPDRFSGSGSGTDFTLKISRVEAEDVGVYYCWQGTHFPYTFGGGTKVEIKRTVAAPSVFIFPPSDEQLKSGTASVVCLLNNFYPREAKVQWKVDNALQSGNSQESVTEQDSKDSTYSLSSTLTLSKADYEKHKVYACEVTHQGLSSPVTKSFNRGEC

SEQ ID NO: 279 - protein, 732 aa, Artificial Sequence
  Third Polypeptide Chain of DART G
QVQLVQSGAEVKKPGASVKVSCKASGYTFTNYGMNWVRQAPGQGLEWMGWINTYTGESTYADDFEGRFVFSMDTSASTAYLQISSLKAEDTAVYYCARESLYDYYSMDYWGQGTTVTVSSASTKGPSVFPLAPSSKSTSGGTAALGCLVKDYFPEPVTVSWNSGALTSGVHTFPAVLQSSGLYSLSSVVTVPSSSLGTQTYICNVNHKPSNTKVDKRVEPKSCDKTHTCPPCPAPEAAGGPSVFLFPPKPKDTLYITREPEVTCVVVDVSHEDPEVKFNWYVDGVEVHNAKTKPREEQYNSTYRVVSVLTVLHQDWLNGKEYKCKVSNKALPAPIEKTISKAKGQPREPQVYTLPPSREEMTKNQVSLWCLVKGFYPSDIAVEWESNGQPENNYKTTPPVLDSDGSFFLYSKLTVDKSRWQQGNVFSCSVMHEALHNHYTQKSLSLSPGGGGSGGGSGGGEIVLTQSPATLSLSPGERATLSCRASESVDNYGMSFMNWFQQKPGQPPKLLIHAASNQGSGVPSRFSGSGSGTDFTLTISSLEPEDFAVYFCQQSKEVPYTFGGGTKVEIKGGGSGGGGQVQLVQSGAEVKKPGASVKVSCKASGYSFTSYWMNWVRQAPGQGLEWIGVIHPSDSETWLDQKFKDRVTITVDKSTSTAYMELSSLRSEDTAVYYCAREHYGTSPFAYWGQGTLVTVSSGGCGGGEVAALEKEVAALEKEVAALEKEVAALEK

SEQ ID NO: 280 - protein, 272 aa, Artificial Sequence
  Fourth Polypeptide Chain of DART G
EIVLTQSPATLSLSPGERATLSCRASESVDNYGMSFMNWFQQKPGQPPKLLIHAASNQGSGVPSRFSGSGSGTDFTLTISSLEPEDFAVYFCQQSKEVPYTFGGGTKVEIKGGGSGGGGQVQLVQSGAEVKKPGASVKVSCKASGYSFTSYWMNWVRQAPGQGLEWIGVIHPSDSETWLDQKFKDRVTITVDKSTSTAYMELSSLRSEDTAVYYCAREHYGTSPFAYWGQGTLVTVSSGGCGGGKVAALKEKVAALKEKVAALKEKVAALKE

SEQ ID NO: 281 - protein, 503 aa, Artificial Sequence
  First Polypeptide Chain of DART H
EIVLTQSPATLSLSPGERATLSCRASESVDNYGMSFMNWFQQKPGQPPKLLIHAASNQGSGVPSRFSGSGSGTDFTLTISSLEPEDFAVYFCQQSKEVPYTFGGGTKVEIKGGGSGGGGQVQLVQSGAEVKKPGASVKVSCKASGYTFTNYGMNWVRQAPGQGLEWMGWINTYTGESTYADDFEGRFVFSMDTSASTAYLQISSLKAEDTAVYYCARESLYDYYSMDYWGQGTTVTVSSGGCGGGEVAALEKEVAALEKEVAALEKEVAALEKGGGDKTHTCPPCPAPEAAGGPSVFLFPPKPKDTLMISRTPEVTCVVVDVSHEDPEVKFNWYVDGVEVHNAKTKPREEQYNSTYRVVSVLTVLHQDWLNGKEYKCKVSNKALPAPIEKTISKAKGQPREPQVYTLPPSREEMTKNQVSLWCLVKGFYPSDIAVEWESNGQPENNYKTTPPVLDSDGSFFLYSKLTVDKSRWQQGNVFSCSVMHEALHNHYTQKSLSLSPGK

SEQ ID NO: 282 - protein, 273 aa, Artificial Sequence
  Second Polypeptide Chain of DART H
DIVMTQTPLSLSVTPGQPASISCKSSQSLLHSDAKTYLNWLLQKPGQPPERLIYLVSELDSGVPDRFSGSGSGTDFTLKISRVEAEDVGVYYCWQGTHFPYTFGGGTKVEIKGGGSGGGGQVQLVQSGAEVKKPGASVKVSCKASGYSFTSYWMNWVRQAPGQGLEWIGVIHPSDSETWLDQKFKDRVTITVDKSTSTAYMELSSLRSEDTAVYYCAREHYGTSPFAYWGQGTLVTVSSGGCGGGKVAALKEKVAALKEKVAALKEKVAALKE

SEQ ID NO: 283 - protein, 227 aa, Artificial Sequence
  Third Polypeptide Chain of DART H
DKTHTCPPCPAPEAAGGPSVFLFPPKPKDTLMISRTPEVTCVVVDVSHEDPEVKFNWYVDGVEVHNAKTKPREEQYNSTYRVVSVLTVLHQDWLNGKEYKCKVSNKALPAPIEKTISKAKGQPREPQVYTLPPSREEMTKNQVSLSCAVKGFYPSDIAVEWESNGQPENNYKTTPPVLDSDGSFFLVSKLTVDKSRWQQGNVFSCSVMHEALHNRYTQKSLSLSPGK

SEQ ID NO: 284 - protein, 563 aa, Artificial Sequence
  First and Third Polypeptide Chains of DART 1
EIVLTQSPATLSLSPGERATLSCRASQSISSYLAWYQQKPGQAPRLLIYDASNRATGIPARFSGSGSGTDFTLTISSLEPEDFAVYYCQQRSNWPLTFGQGTNLEIKGGGSGGGGQVQLVESGGGVVQPGRSLRLDCKASGITFSNSGMHWVRQAPGKGLEWVAVIWYDGSKRYYADSVKGRFTISRDNSKNTLFLQMNSLRAEDTAVYYCATNDDYWGQGTLVTVSSLGGGSGASTKGPSVFPLAPSSKSTSGGTAALGCLVKDYFPEPVTVSWNSGALTSGVHTFPAVLQSSGLYSLSSVVTVPSSSLGTQTYICNVNHKPSNTKVDKRVEPKSCDKTHTCPPCPAPEAAGGPSVFLFPPKPKDTLYITREPEVTCVVVDVSHEDPEVKFNWYVDGVEVHNAKTKPREEQYNSTYRVVSVLTVLHQDWLNGKEYKCKVSNKALPAPIEKTISKAKGQPREPQVYTLPPSREEMTKNQVSLTCLVKGFYPSDIAVEWESNGQPENNYKTTPPVLDSDGSFFLYSKLTVDKSRWQQGNVFSCSVMHEALHNHYTQKSLSLSPG

SEQ ID NO: 285 - protein, 348 aa, Artificial Sequence
  Second and Fourth Polypeptide Chains of DART 1
EIVLTQSPATLSLSPGERATLSCRASQSVSSYLAWYQQKPGQAPRLLIYDASNRATGIPARFSGSGSGTDFTLTISSLEPEDFAVYYCQQSSNWPRTFGQGTKVEIKGGGSGGGGQVQLQQWGAGLLKPSETLSLTCAVYGGSFSDYYWNWIRQPPGKGLEWIGEINHNGNTNSNPSLKSRVTLSLDTSKNQFSLKLRSVTAADTAVYYCAFGYSDYEYNWFDPWGQGTLVTVSSLGGGSGRTVAAPSVFIFPPSDEQLKSGTASVVCLLNNFYPREAKVQWKVDNALQSGNSQESVTEQDSKDSTYSLSSTLTLSKADYEKHKVYACEVTHQGLSSPVTKSFNRGEC

SEQ ID NO: 286 - protein, 448 aa, Artificial Sequence
  First Polypeptide Chain of BSAB A
QVQLVQSGAEVKKPGASVKVSCKASGYSFTSYWMNWVRQAPGQGLEWIGVIHPSDSETWLDQKFKDRVTITVDKSTSTAYMELSSLRSEDTAVYYCAREHYGTSPFAYWGQGTLVTVSSASTKGPSVFPLAPSSKSTSGGTAALGCLVKDYFPEPVTVSWNSGALTSGVHTFPAVLQSSGLYSLSSVVTVPSSSLGTQTYICNVNHKPSNTKVDKRVEPKSCEKTHTCPECPAPEAAGGPSVFLFPPKPKDTLMISRTPEVTCVVVDVSHEDPEVKFNWYVDGVEVHNAKTKPREEQYNSTYRVVSVLTVLHQDWLNGKEYKCKVSNKALPAPIEKTISKAKGQPREPQVYTLPPSREEMTKNQVSLTCEVKGFYPSDIAVEWESNGQPENNYKTTPPVLDSDGSFFLYSKLTVDKSRWQQGNVFSCSVMHEALHNHYTQKSLSLSPG

SEQ ID NO: 287 - protein, 218 aa, Artificial Sequence; identical to SEQ ID NO: 264
  Second Polypeptide Chain of BSAB A

SEQ ID NO: 288 - protein, 449 aa, Artificial Sequence
  Third Polypeptide Chain of BSAB A
QVQLVQSGAEVKKPGASVKVSCKASGYTFTNYGMNWVRQAPGQGLEWMGWINTYTGESTYADDFEGRFVFSMDTSASTAYLQISSLKAEDTAVYYCARESLYDYYSMDYWGQGTTVTVSSASTKGPSVFPLAPSSKSTSGGTAALGCLVKDYFPEPVTVSWNSGALTSGVHTFPAVLQSSGLYSLSSVVTVPSSSLGTQTYICNVNHKPSNTKVDKRVEPKSCRKTHTCPRCPAPEAAGGPSVFLFPPKPKDTLMISRTPEVTCVVVDVSHEDPEVKFNWYVDGVEVHNAKTKPREEQYNSTYRVVSVLTVLHQDWLNGKEYKCKVSNKALPAPIEKTISKAKGQPREPQVYTLPPSREEMTKNQVSLTCLVKGFYPSDIAVEWESNGQPENNYKTTPPVLDSDGSFFLYSRLTVDKSRWQQGNVFSCSVMHEALHNHYTQKSLSLSPG

SEQ ID NO: 289 - protein, 219 aa, Artificial Sequence; identical to SEQ ID NO: 278
  Fourth Polypeptide Chain of BSAB A

SEQ ID NO: 290 - protein, 496 aa, Artificial Sequence
  First and Third Polypeptide Chains of DART I
DIQMTQSPSSLSASVGDRVTITCRASQDVSSVVAWYQQKPGKAPKLLIYSASYRYTGVPSRFSGSGSGTDFTLTISSLQPEDFATYYCQQHYSTPWTFGGGTKLEIKGGGSGGGGQVQLVQSGAEVKKPGASVKVSCKASGYSFTSYWMNWVRQAPGQGLEWIGVIHPSDSETWLDQKFKDRVTITVDKSTSTAYMELSSLRSEDTAVYYCAREHYGTSPFAYWGQGTLVTVSSGGCGGGEVAACEKEVAALEKEVAALEKEVAALEKESKYGPPCPPCPAPEFLGGPSVFLFPPKPKDTLYITREPEVTCVVVDVSQEDPEVQFNWYVDGVEVHNAKTKPREEQFNSTYRVVSVLTVLHQDWLNGKEYKCKVSNKGLPSSIEKTISKAKGQPREPQVYTLPPSQEEMTKNQVSLTCLVKGFYPSDIAVEWESNGQPENNYKTTPPVLDSDGSFFLYSRLTVDKSRWQEGNVFSCSVMHEALHNHYTQKSLSLSLG

SEQ ID NO: 291 - protein, 271 aa, Artificial Sequence
  Second and Fourth Polypeptide Chains of DART I
EIVLTQSPATLSLSPGERATLSCRASESVDNYGMSFMNWFQQKPGQPPKLLIHAASNQGSGVPSRFSGSGSGTDFTLTISSLEPEDFAVYFCQQSKEVPYTFGGGTKVEIKGGGSGGGGQVQLVQSGAEVKKPGASVKVSCKASGYTFTDYNMDWVRQAPGQGLEWMGDINPDNGVTIYNQKFEGRVTMTTDTSTSTAYMELRSLRSDDTAVYYCAREADYFYFDYWGQGTTLTVSSGGCGGGKVAACKEKVAALKEKVAALKEKVAALKE

SEQ ID NO: 292 - protein, 566 aa, Artificial Sequence
  First and Third Polypeptide Chains of DART J
DIQMTQSPSSLSASVGDRVTITCRASQDVSSVVAWYQQKPGKAPKLLIYSASYRYTGVPSRFSGSGSGTDFTLTISSLQPEDFATYYCQQHYSTPWTFGGGTKLEIKGGGSGGGGQVQLVQSGAEVKKPGASVKVSCKASGYSFTSYWMNWVRQAPGQGLEWIGVIHPSDSETWLDQKFKDRVTITVDKSTSTAYMELSSLRSEDTAVYYCAREHYGTSPFAYWGQGTLVTVSSLGGGSGASTKGPSVFPLAPCSRSTSESTAALGCLVKDYFPEPVTVSWNSGALTSGVHTFPAVLQSSGLYSLSSVVTVPSSSLGTKTYTCNVDHKPSNTKVDKRVESKYGPPCPPCPAPEFLGGPSVFLFPPKPKDTLYITREPEVTCVVVDVSQEDPEVQFNWYVDGVEVHNAKTKPREEQFNSTYRVVSVLTVLHQDWLNGKEYKCKVSNKGLPSSIEKTISKAKGQPREPQVYTLPPSQEEMTKNQVSLTCLVKGFYPSDIAVEWESNGQPENNYKTTPPVLDSDGSFFLYSRLTVDKSRWQEGNVFSCSVMHEALHNHYTQKSLSLSLG

SEQ ID NO: 293 - protein, 350 aa, Artificial Sequence
  Second and Fourth Polypeptide Chains of DART J
EIVLTQSPATLSLSPGERATLSCRASESVDNYGMSFMNWFQQKPGQPPKLLIHAASNQGSGVPSRFSGSGSGTDFTLTISSLEPEDFAVYFCQQSKEVPYTFGGGTKVEIKGGGSGGGGQVQLVQSGAEVKKPGASVKVSCKASGYTFTDYNMDWVRQAPGQGLEWMGDINPDNGVTIYNQKFEGRVTMTTDTSTSTAYMELRSLRSDDTAVYYCAREADYFYFDYWGQGTTLTVSSLGGGSGRTVAAPSVFIFPPSDEQLKSGTASVVCLLNNFYPREAKVQWKVDNALQSGNSQESVTEQDSKDSTYSLSSTLTLSKADYEKHKVYACEVTHQGLSSPVTKSFNRGEC

SEQ ID NO: 294 - protein, 118 aa, Artificial Sequence
  VH Domain of hLAG-3 mAb 6 VH1
QVQLVQSGAEVKKPGASVKVSCKASGYTFTDYNMDWVRQAPGQGLEWMGDINPDNGVTIYNQKFEGRVTMTTDTSTSTAYMELRSLRSDDTAVYYCAREADYFYFDYWGQGTTLTVSS

SEQ ID NO: 295 - protein, 118 aa, Artificial Sequence
  VH Domain of hLAG-3 mAb 6 VH2
EVQLVESGGGLVKPGGSLRLSCAASGFTFSDYNMDWVRQAPGKGLEWVSDINPDNGVTIYNQKFEGRFTISRDNAKNSLYLQMNSLRAEDTAVYYCAREADYFYFDYWGQGTTLTVSS

SEQ ID NO: 296 - protein, 107 aa, Artificial Sequence
  VL Domain of hLAG-3 mAb 6 VL1
DIQMTQSPSSLSASVGDRVTITCRASQDVSSVVAWYQQKPGKAPKLLIYSASYRYTGVPSRFSGSGSGTDFTLTISSLQPEDFATYYCQQHYSTPWTFGGGTKLEIK

SEQ ID NO: 297 - protein, 107 aa, Artificial Sequence
  VL Domain of hLAG-3 mAb 6 VL2
DIVMTQSPSSLSASVGDRVTITCRASQDVSSVVAWYQQKPGKAPKLLIYSASYRYTGVPDRFSGSGSGTDFTFTISSLQPEDIAVYYCQQHYSTPWTFGGGTKLEIK

SEQ ID NO: 298 - protein, 11 aa, Artificial Sequence
  CDRL1 of the VL Domain of hLAG-3 mAb 6 VL1 and VL2
RASQDVSSVVA